European Patent Application EP 4 122 953 A1, published January 25, 2023. Title: FUSION PROTEIN COMPRISING IL-2 PROTEIN AND CD80 PROTEIN FRAGMENT OR MUTEIN THEREOF AND USE THEREOF. Applicant: GI Innovation, Inc. The sequence listing filed with the application follows.

SEQUENCE LISTING (115 sequences)

SEQ ID NO: 1 - protein, 25 aa, Artificial Sequence
  signal peptide (TPA)
MDAMLRGLCCVLLLCGAVFVSPSHA

SEQ ID NO: 2 - protein, 208 aa, Artificial Sequence [sequence omitted]

SEQ ID NO: 3 - protein, 30 aa, Artificial Sequence
  hinge
GSGGGGSGGGGSGGGGSAESKYGPPCPPCP

SEQ ID NO: 4 - protein, 216 aa, Artificial Sequence
  immunoglobulin fc
APEAAGGPSVFLFPPKPKDQLMISRTPEVTCVVVDVSQEDPEVQFNWYVDGVEVHNAKTKPREEQFNSTYRVVSVLTVLHQDWLNGKEYKCKVSNKGLPSSIEKTISKAKGQPREPQVYTLPPSQEEMTKNQVSLTCLVKGFYPSDIAVEWESNGQPENNYKTTPPVLDSDGSFFLYSRLTVDKSRWQEGNVFSCSVLHEALHNHYTQKSLSLSLG

SEQ ID NO: 5 - protein, 5 aa, Artificial Sequence
  linker
GGGGS

SEQ ID NO: 6 - protein, 133 aa, Artificial Sequence
  hIL-2M
APTSSSTKKTQLQLEHLLLDLQMILNGINNYKNPKLTAMLTAKFYMPKKATELKHLQCLEEELKPLEEVLNLAQSKNFHLRPRDLISNINVIVLELKGSETTFMCEYADETATIVEFLNRWITFCQSIISTLT

SEQ ID NO: 7 - protein, 617 aa, Artificial Sequence
  fusion protein comprising variants of IL-2 and fragments of CD80
MDAMLRGLCCVLLLCGAVFVSPSHAVIHVTKEVKEVATLSCGHNVSVEELAQTRIYWQKEKKMVLTMMSGDMNIWPEYKNRTIFDITNNLSIVILALRPSDEGTYECVVLKYEKDAFKREHLAEVTLSVKADFPTPSISDFEIPTSNIRRIICSTSGGFPEPHLSWLENGEELNAINTTVSQDPETELYAVSSKLDFNMTTNHSFMCLIKYGHLRVNQTFNWNTTKQEHFPDNGSGGGGSGGGGSGGGGSAESKYGPPCPPCPAPEAAGGPSVFLFPPKPKDQLMISRTPEVTCVVVDVSQEDPEVQFNWYVDGVEVHNAKTKPREEQFNSTYRVVSVLTVLHQDWLNGKEYKCKVSNKGLPSSIEKTISKAKGQPREPQVYTLPPSQEEMTKNQVSLTCLVKGFYPSDIAVEWESNGQPENNYKTTPPVLDSDGSFFLYSRLTVDKSRWQEGNVFSCSVLHEALHNHYTQKSLSLSLGGGGGSAPTSSSTKKTQLQLEHLLLDLQMILNGINNYKNPKLTAMLTAKFYMPKKATELKHLQCLEEELKPLEEVLNLAQSKNFHLRPRDLISNINVIVLELKGSETTFMCEYADETATIVEFLNRWITFCQSIISTLT

SEQ ID NO: 8 - DNA, 1857 bp, Artificial Sequence
  nucleotiedes coding fusion protein (GI101)
atggatgctatgctgagaggcctgtgttgcgtgctgctgctgtgtggcgctgtgttcgtgtctccttctcacgctgtgatccacgtgaccaaagaagtgaaagaggtcgccacactgtcctgcggccacaacgtttcagtggaagaactggcccagaccaggatctactggcagaaagaaaagaaaatggtgctgaccatgatgtccggcgacatgaacatctggcctgagtacaagaaccggaccatcttcgacatcaccaacaacctgtccatcgtgattctggccctgaggccttctgatgagggcacctatgagtgcgtggtgctgaagtacgagaaggacgccttcaagcgcgagcacctggctgaagtgacactgtccgtgaaggccgactttcccacaccttccatctccgacttcgagatccctacctccaacatccggcggatcatctgttctacctctggcggctttcctgagcctcacctgtcttggctggaaaacggcgaggaactgaacgccatcaacaccaccgtgtctcaggaccccgaaaccgagctgtacgctgtgtcctccaagctggacttcaacatgaccaccaaccacagcttcatgtgcctgattaagtacggccacctgagagtgaaccagaccttcaactggaacaccaccaagcaagagcacttccctgacaatggatctggcggcggaggttctggcggaggtggaagcggaggcggaggatctgctgagtctaagtatggccctccttgtcctccatgtcctgctccagaagctgctggcggaccctctgtgttcctgtttcctccaaagcctaaggaccagctcatgatctctcggacacccgaagtgacctgcgtggtggtggatgtgtctcaagaggaccctgaggtgcagttcaattggtacgtggacggcgtggaagtgcacaacgccaagaccaagcctagagaggaacagttcaactccacctacagagtggtgtccgtgctgaccgtgctgcaccaggattggctgaacggcaaagagtacaagtgcaaggtgtccaacaagggcctgccttccagcatcgaaaagaccatctccaaggctaagggccagcctagggaaccccaggtttacaccctgcctccaagccaagaggaaatgaccaagaaccaggtgtccctgacctgcctggtcaagggcttctacccttccgacattgccgtggaatgggagtccaatggccagcctgagaacaactacaagaccacacctcctgtgctggactccgacggctccttctttctgtactctcgcctgaccgtggacaagtctagatggcaagagggcaacgtgttctcctgctctgtgctgcacgaggccctgcacaatcactacacccagaagtccctgtctctgtctcttggaggtggtggcggttctgcccctaccagctcctctaccaagaaaacccagctccagttggagcatctgctgctggacctccagatgattctgaacgggatcaacaactataagaaccccaagctgaccgccatgctgaccgctaagttctacatgcccaagaaggccaccgagctgaagcacctccagtgcctggaagaagaactgaagcccctggaagaggtgctgaatctggcccagtccaagaacttccacctgaggccacgggacctgatcagcaacatcaacgtgatcgtgctggaactgaagggctccgagacaacctttatgtgcgagtacgccgacgagacagccaccatcgtggaatttctgaaccggtggatcaccttctgccagagcatcatctccacactgacctgatga

SEQ ID NO: 9 - protein, 592 aa, Artificial Sequence
  fusion protein (GI101)
VIHVTKEVKEVATLSCGHNVSVEELAQTRIYWQKEKKMVLTMMSGDMNIWPEYKNRTIFDITNNLSIVILALRPSDEGTYECVVLKYEKDAFKREHLAEVTLSVKADFPTPSISDFEIPTSNIRRIICSTSGGFPEPHLSWLENGEELNAINTTVSQDPETELYAVSSKLDFNMTTNHSFMCLIKYGHLRVNQTFNWNTTKQEHFPDNGSGGGGSGGGGSGGGGSAESKYGPPCPPCPAPEAAGGPSVFLFPPKPKDQLMISRTPEVTCVVVDVSQEDPEVQFNWYVDGVEVHNAKTKPREEQFNSTYRVVSVLTVLHQDWLNGKEYKCKVSNKGLPSSIEKTISKAKGQPREPQVYTLPPSQEEMTKNQVSLTCLVKGFYPSDIAVEWESNGQPENNYKTTPPVLDSDGSFFLYSRLTVDKSRWQEGNVFSCSVLHEALHNHYTQKSLSLSLGGGGGSAPTSSSTKKTQLQLEHLLLDLQMILNGINNYKNPKLTAMLTAKFYMPKKATELKHLQCLEEELKPLEEVLNLAQSKNFHLRPRDLISNINVIVLELKGSETTFMCEYADETATIVEFLNRWITFCQSIISTLT

SEQ ID NO: 10 - protein, 133 aa, Artificial Sequence [sequence omitted]

SEQ ID NO: 11 - protein, 288 aa, Artificial Sequence
  CD80
MGHTRRQGTSPSKCPYLNFFQLLVLAGLSHFCSGVIHVTKEVKEVATLSCGHNVSVEELAQTRIYWQKEKKMVLTMMSGDMNIWPEYKNRTIFDITNNLSIVILALRPSDEGTYECVVLKYEKDAFKREHLAEVTLSVKADFPTPSISDFEIPTSNIRRIICSTSGGFPEPHLSWLENGEELNAINTTVSQDPETELYAVSSKLDFNMTTNHSFMCLIKYGHLRVNQTFNWNTTKQEHFPDNLLPSWAITLISVNGIFVICCLTYCFAPRCRERRRNERLRRESVRPV

SEQ ID NO: 12 - protein, 215 aa, Artificial Sequence
  modified Fc
SHTQPLGVFLFPPKPKDTLMISRTPEVTCVVVDVSQEDPEVQFNWYVDGVEVHNAKTKPREEQFNSTYRVVSVLTVLHQDWLNGKEYKCKVSNKGLPSSIEKTISKAKGQPREPQVYTLPPSQEEMTKNQVSLTCLVKGFYPSDIAVEWESNGQPENNYKTTPPVLDSDGSFFLYSRLTVDKSRWQEGNVFSCSVMHEALHNHYTQKSLSLSLGK

SEQ ID NO: 13 - protein, 306 aa, Artificial Sequence
  mCD80
MACNCQLMQDTPLLKFPCPRLILLFVLLIRLSQVSSDVDEQLSKSVKDKVLLPCRYNSPHEDESEDRIYWQKHDKVVLSVIAGKLKVWPEYKNRTLYDNTTYSLIILGLVLSDRGTYSCVVQKKERGTYEVKHLALVKLSIKADFSTPNITESGNPSADTKRITCFASGGFPKPRFSWLENGRELPGINTTISQDPESELYTISSQLDFNTTRNHTIKCLIKYGDAHVSEDFTWEKPPEDPPDSKNTLVLFGAGFGAVITVVVIVVIIKCFCKHRSCFRRNEASRETNNSLTFGPEEALAEQTVFL

SEQ ID NO: 14 - DNA, 1848 bp, Artificial Sequence
  nucleotiedes coding fusion protein (mGI101)
atggatgctatgctgagaggcctgtgttgcgtgctgctgctgtgtggcgctgtgttcgtgtctccttctcacgctgtggacgagcagctctccaagtccgtgaaggataaggtcctgctgccttgccggtacaactctcctcacgaggacgagtctgaggaccggatctactggcagaaacacgacaaggtggtgctgtccgtgatcgccggaaagctgaaagtgtggcctgagtacaagaacaggaccctgtacgacaacaccacctacagcctgatcatcctgggcctcgtgctgagcgatagaggcacctattcttgcgtggtgcagaagaaagagcggggcacctacgaagtgaagcacctggctctggtcaagctgtccatcaaggccgacttcagcacccctaacatcaccgagtctggcaacccttccgccgacaccaagagaatcacctgtttcgcctctggcggcttccctaagcctcggttctcttggctggaaaacggcagagagctgcccggcatcaataccaccatttctcaggacccagagtccgagctgtacaccatctccagccagctcgactttaacaccaccagaaaccacaccatcaagtgcctgattaagtacggcgacgcccacgtgtccgaggactttacttgggagaaacctcctgaggaccctcctgactctggatctggcggcggaggttctggcggaggtggaagcggaggcggaggatctgctgagtctaagtatggccctccttgtcctccatgtcctgctccagaagctgctggcggaccctctgtgttcctgtttcctccaaagcctaaggaccagctcatgatctctcggacccctgaagtgacctgcgtggtggtggatgtgtctcaagaggaccctgaggtgcagttcaattggtacgtggacggcgtggaagtgcacaacgccaagaccaagcctagagaggaacagttcaactccacctatagagtggtgtccgtgctgaccgtgctgcaccaggattggctgaacggcaaagagtacaagtgcaaggtgtccaacaagggcctgccttccagcatcgaaaagaccatcagcaaggctaagggccagcctagggaaccccaggtttacaccctgcctccaagccaagaggaaatgaccaagaaccaggtgtccctgacctgcctggtcaagggcttctacccttccgacattgccgtggaatgggagtccaatggccagcctgagaacaactacaagaccacacctcctgtgctggactccgacggctccttctttctgtactctcgcctgaccgtggacaagtctaggtggcaagagggcaacgtgttctcctgctctgtgctgcacgaggctctgcacaaccactacacccagaagtccctgtctctgtctcttggaggtggtggcggttctgcccctacctccagctctaccaagaaaacccagctccagttggagcatctgctgctggacctccagatgatcctgaatggcatcaacaattacaagaaccccaagctgaccgccatgctgaccgctaagttctacatgcccaagaaggccaccgagctgaagcacttgcagtgcctggaagaggaactgaagcccctggaagaagtgctgaatctggcccagtccaagaacttccacctgaggcctagggacctgatctccaacatcaacgtgatcgtgctggaactgaaaggctccgagacaaccttcatgtgcgagtacgccgacgagacagccaccatcgtggaatttctgaaccggtggatcaccttctgccagagcatcatctccacactgacc

SEQ ID NO: 15 - protein, 616 aa, Artificial Sequence
  fusion protein (mGI101)
MDAMLRGLCCVLLLCGAVFVSPSHAVDEQLSKSVKDKVLLPCRYNSPHEDESEDRIYWQKHDKVVLSVIAGKLKVWPEYKNRTLYDNTTYSLIILGLVLSDRGTYSCVVQKKERGTYEVKHLALVKLSIKADFSTPNITESGNPSADTKRITCFASGGFPKPRFSWLENGRELPGINTTISQDPESELYTISSQLDFNTTRNHTIKCLIKYGDAHVSEDFTWEKPPEDPPDSGSGGGGSGGGGSGGGGSAESKYGPPCPPCPAPEAAGGPSVFLFPPKPKDQLMISRTPEVTCVVVDVSQEDPEVQFNWYVDGVEVHNAKTKPREEQFNSTYRVVSVLTVLHQDWLNGKEYKCKVSNKGLPSSIEKTISKAKGQPREPQVYTLPPSQEEMTKNQVSLTCLVKGFYPSDIAVEWESNGQPENNYKTTPPVLDSDGSFFLYSRLTVDKSRWQEGNVFSCSVLHEALHNHYTQKSLSLSLGGGGGSAPTSSSTKKTQLQLEHLLLDLQMILNGINNYKNPKLTAMLTAKFYMPKKATELKHLQCLEEELKPLEEVLNLAQSKNFHLRPRDLISNINVIVLELKGSETTFMCEYADETATIVEFLNRWITFCQSIISTLT

SEQ ID NO: 16 - DNA, 1437 bp, Artificial Sequence
  nucleotiedes coding fusion protein (GI101C1)
atggatgctatgctgagaggcctgtgttgcgtgctgctgctgtgtggcgctgtgttcgtgtctccttctcacgctgtgatccacgtgaccaaagaagtgaaagaggtcgccacactgtcctgcggccacaacgtttcagtggaagaactggcccagaccaggatctactggcagaaagaaaagaaaatggtgctgaccatgatgtccggcgacatgaacatctggcctgagtacaagaaccggaccatcttcgacatcaccaacaacctgtccatcgtgattctggccctgaggccttctgatgagggcacctatgagtgcgtggtgctgaagtacgagaaggacgccttcaagcgcgagcacctggctgaagtgacactgtccgtgaaggccgactttcccacaccttccatctccgacttcgagatccctacctccaacatccggcggatcatctgttctacctctggcggctttcctgagcctcacctgtcttggctggaaaacggcgaggaactgaacgccatcaacaccaccgtgtctcaggaccccgaaaccgagctgtacgctgtgtcctccaagctggacttcaacatgaccaccaaccacagcttcatgtgcctgattaagtacggccacctgagagtgaaccagaccttcaactggaacaccaccaagcaagagcacttccctgacaatggatctggcggcggaggttctggcggaggtggaagcggaggcggaggatctgctgagtctaagtatggccctccttgtcctccatgtcctgctccagaagctgctggcggaccctctgtgttcctgtttcctccaaagcctaaggaccagctcatgatctctcggacacccgaagtgacctgcgtggtggtggatgtgtctcaagaggaccctgaggtgcagttcaattggtacgtggacggcgtggaagtgcacaacgccaagaccaagcctagagaggaacagttcaactccacctacagagtggtgtccgtgctgaccgtgctgcaccaggattggctgaacggcaaagagtacaagtgcaaggtgtccaacaagggcctgccttccagcatcgaaaagaccatctccaaggctaagggccagcctagggaaccccaggtttacaccctgcctccaagccaagaggaaatgaccaagaaccaggtgtccctgacctgcctggtcaagggcttctacccttccgacattgccgtggaatgggagtccaatggccagcctgagaacaactacaagaccacacctcctgtgctggactccgacggctccttctttctgtactctcgcctgaccgtggacaagtctaggtggcaagagggcaacgtgttctcctgctctgtgctgcacgaggccctgcacaatcactacacccagaagtccctgtctctgtccctgggc

SEQ ID NO: 17 - protein, 454 aa, Artificial Sequence
  fusion protein (GI101C1)
VIHVTKEVKEVATLSCGHNVSVEELAQTRIYWQKEKKMVLTMMSGDMNIWPEYKNRTIFDITNNLSIVILALRPSDEGTYECVVLKYEKDAFKREHLAEVTLSVKADFPTPSISDFEIPTSNIRRIICSTSGGFPEPHLSWLENGEELNAINTTVSQDPETELYAVSSKLDFNMTTNHSFMCLIKYGHLRVNQTFNWNTTKQEHFPDNGSGGGGSGGGGSGGGGSAESKYGPPCPPCPAPEAAGGPSVFLFPPKPKDQLMISRTPEVTCVVVDVSQEDPEVQFNWYVDGVEVHNAKTKPREEQFNSTYRVVSVLTVLHQDWLNGKEYKCKVSNKGLPSSIEKTISKAKGQPREPQVYTLPPSQEEMTKNQVSLTCLVKGFYPSDIAVEWESNGQPENNYKTTPPVLDSDGSFFLYSRLTVDKSRWQEGNVFSCSVLHEALHNHYTQKSLSLSLG

SEQ ID NO: 18 - DNA, 1176 bp, Artificial Sequence
  nucleotiedes coding fusion protein (GI101C2)
atggatgctatgctgagaggcctgtgttgcgtgctgctgctgtgtggcgctgtgttcgtgtctccatctcacgccgctgagtctaagtacggccctccttgtcctccatgtcctgctccagaagctgctggcggaccctctgtgttcctgtttcctccaaagcctaaggaccagctcatgatctctcggacccctgaagtgacctgcgtggtggtggatgtgtctcaagaggaccctgaggtgcagttcaattggtacgtggacggcgtggaagtgcacaacgccaagaccaagcctagagaggaacagttcaactccacctacagagtggtgtccgtgctgaccgtgctgcaccaggattggctgaacggcaaagagtacaagtgcaaggtgtccaacaagggcctgccttccagcatcgaaaagaccatctccaaggctaagggccagcctagggaaccccaggtttacaccctgcctccaagccaagaggaaatgaccaagaaccaggtgtccctgacctgcctggtcaagggcttctacccttccgacattgccgtggaatgggagtccaatggccagcctgagaacaactacaagaccacacctcctgtgctggactccgacggctccttctttctgtactctcgcctgaccgtggacaagtctaggtggcaagagggcaacgtgttctcctgctctgtgctgcacgaggccctgcacaatcactacacccagaagtccctgtctctgtctcttggcggaggcggaggatctgctcctacctccagctccaccaagaaaacccagctccagttggagcatctgctgctggacctccagatgatcctgaatggcatcaacaattacaagaaccccaagctgaccgccatgctgaccgctaagttctacatgcccaagaaggccaccgagctgaagcacctccagtgcctggaagaggaactgaagcccctggaagaagtgctgaatctggcccagtccaagaacttccacctgaggcctagggacctgatctccaacatcaacgtgatcgtgctggaactgaaaggctccgagacaaccttcatgtgcgagtacgccgacgagacagccaccatcgtggaatttctgaaccggtggatcaccttctgccagtccatcatctccacactgacc

SEQ ID NO: 19 - protein, 367 aa, Artificial Sequence
  fusion protein (GI101C2)
AESKYGPPCPPCPAPEAAGGPSVFLFPPKPKDQLMISRTPEVTCVVVDVSQEDPEVQFNWYVDGVEVHNAKTKPREEQFNSTYRVVSVLTVLHQDWLNGKEYKCKVSNKGLPSSIEKTISKAKGQPREPQVYTLPPSQEEMTKNQVSLTCLVKGFYPSDIAVEWESNGQPENNYKTTPPVLDSDGSFFLYSRLTVDKSRWQEGNVFSCSVLHEALHNHYTQKSLSLSLGGGGGSAPTSSSTKKTQLQLEHLLLDLQMILNGINNYKNPKLTAMLTAKFYMPKKATELKHLQCLEEELKPLEEVLNLAQSKNFHLRPRDLISNINVIVLELKGSETTFMCEYADETATIVEFLNRWITFCQSIISTLT

SEQ ID NO: 20 - DNA, 1434 bp, Artificial Sequence
  nucleotiedes coding fusion protein (mGI101C1)
atggatgctatgctgagaggcctgtgttgcgtgctgctgctgtgtggcgctgtgttcgtgtctccttctcacgctgtggacgagcagctctccaagtccgtgaaggataaggtcctgctgccttgccggtacaactctcctcacgaggacgagtctgaggaccggatctactggcagaaacacgacaaggtggtgctgtccgtgatcgccggaaagctgaaagtgtggcctgagtacaagaacaggaccctgtacgacaacaccacctacagcctgatcatcctgggcctcgtgctgagcgatagaggcacctattcttgcgtggtgcagaagaaagagcggggcacctacgaagtgaagcacctggctctggtcaagctgtccatcaaggccgacttcagcacccctaacatcaccgagtctggcaacccttccgccgacaccaagagaatcacctgtttcgcctctggcggcttccctaagcctcggttctcttggctggaaaacggcagagagctgcccggcatcaataccaccatttctcaggacccagagtccgagctgtacaccatctccagccagctcgactttaacaccaccagaaaccacaccatcaagtgcctgattaagtacggcgacgcccacgtgtccgaggactttacttgggagaaacctcctgaggaccctcctgactctggatctggcggcggaggttctggcggaggtggaagcggaggcggaggatctgctgagtctaagtatggccctccttgtcctccatgtcctgctccagaagctgctggcggaccctctgtgttcctgtttcctccaaagcctaaggaccagctcatgatctctcggacccctgaagtgacctgcgtggtggtggatgtgtctcaagaggaccctgaggtgcagttcaattggtacgtggacggcgtggaagtgcacaacgccaagaccaagcctagagaggaacagttcaactccacctatagagtggtgtccgtgctgaccgtgctgcaccaggattggctgaacggcaaagagtacaagtgcaaggtgtccaacaagggcctgccttccagcatcgaaaagaccatcagcaaggctaagggccagcctagggaaccccaggtttacaccctgcctccaagccaagaggaaatgaccaagaaccaggtgtccctgacctgcctggtcaagggcttctacccttccgacattgccgtggaatgggagtccaatggccagcctgagaacaactacaagaccacacctcctgtgctggactccgacggctccttctttctgtactctcgcctgaccgtggacaagtctaggtggcaagagggcaacgtgttctcctgctctgtgctgcacgaggctctgcacaaccactacacccagaagtccctgtctctgtccctgggc

SEQ ID NO: 21 - protein, 478 aa, Artificial Sequence
  fusion protein (mGI101C1)
MDAMLRGLCCVLLLCGAVFVSPSHAVDEQLSKSVKDKVLLPCRYNSPHEDESEDRIYWQKHDKVVLSVIAGKLKVWPEYKNRTLYDNTTYSLIILGLVLSDRGTYSCVVQKKERGTYEVKHLALVKLSIKADFSTPNITESGNPSADTKRITCFASGGFPKPRFSWLENGRELPGINTTISQDPESELYTISSQLDFNTTRNHTIKCLIKYGDAHVSEDFTWEKPPEDPPDSGSGGGGSGGGGSGGGGSAESKYGPPCPPCPAPEAAGGPSVFLFPPKPKDQLMISRTPEVTCVVVDVSQEDPEVQFNWYVDGVEVHNAKTKPREEQFNSTYRVVSVLTVLHQDWLNGKEYKCKVSNKGLPSSIEKTISKAKGQPREPQVYTLPPSQEEMTKNQVSLTCLVKGFYPSDIAVEWESNGQPENNYKTTPPVLDSDGSFFLYSRLTVDKSRWQEGNVFSCSVLHEALHNHYTQKSLSLSLG

SEQ ID NO: 22 - protein, 133 aa, Artificial Sequence
  variants of IL-2 (3M, M45)
APTSSSTKKTQLQLEHLLLDLQMILNGINNYKNPKLTAMLTAKFAMPKKATELKHLQCLEEELKPLEEVLNLAQSKNFHLRPRDLISNINVIVLELKGSETTFMCEYADETATIVEFLNRWITFCQSIISTLT

SEQ ID NO: 23 - protein, 133 aa, Artificial Sequence
  variants of IL-2 (3M, M61)
APTSSSTKKTQLQLEHLLLDLQMILNGINNYKNPKLTAMLTAKFYMPKKATELKHLQCLERELKPLEEVLNLAQSKNFHLRPRDLISNINVIVLELKGSETTFMCEYADETATIVEFLNRWITFCQSIISTLT

SEQ ID NO: 24 - protein, 133 aa, Artificial Sequence
  variants of IL-2 (3M, M72)
APTSSSTKKTQLQLEHLLLDLQMILNGINNYKNPKLTAMLTAKFYMPKKATELKHLQCLEEELKPLEEVLNGAQSKNFHLRPRDLISNINVIVLELKGSETTFMCEYADETATIVEFLNRWITFCQSIISTLT

SEQ ID NO: 25 - DNA, 1851 bp, Artificial Sequence
  nucleotiedes coding fusion protein (GI102-M45)
atggatgctatgctgagaggcctgtgttgcgtgctgctgctgtgtggcgctgtgttcgtgtctccttctcacgctgtgatccacgtgaccaaagaagtgaaagaggtcgccacactgtcctgcggccacaacgtttcagtggaagaactggcccagaccaggatctactggcagaaagaaaagaaaatggtgctgaccatgatgtccggcgacatgaacatctggcctgagtacaagaaccggaccatcttcgacatcaccaacaacctgtccatcgtgattctggccctgaggccttctgatgagggcacctatgagtgcgtggtgctgaagtacgagaaggacgccttcaagcgcgagcacctggctgaagtgacactgtccgtgaaggccgactttcccacaccttccatctccgacttcgagatccctacctccaacatccggcggatcatctgttctacctctggcggctttcctgagcctcacctgtcttggctggaaaacggcgaggaactgaacgccatcaacaccaccgtgtctcaggaccccgaaaccgagctgtacgctgtgtcctccaagctggacttcaacatgaccaccaaccacagcttcatgtgcctgattaagtacggccacctgagagtgaaccagaccttcaactggaacaccaccaagcaagagcacttccctgacaatggatctggcggcggaggttctggcggaggtggaagcggaggcggaggatctgctgagtctaagtatggccctccttgtcctccatgtcctgctccagaagctgctggcggaccctctgtgttcctgtttcctccaaagcctaaggaccagctcatgatctctcggacacccgaagtgacctgcgtggtggtggatgtgtctcaagaggaccctgaggtgcagttcaattggtacgtggacggcgtggaagtgcacaacgccaagaccaagcctagagaggaacagttcaactccacctacagagtggtgtccgtgctgaccgtgctgcaccaggattggctgaacggcaaagagtacaagtgcaaggtgtccaacaagggcctgccttccagcatcgaaaagaccatctccaaggctaagggccagcctagggaaccccaggtttacaccctgcctccaagccaagaggaaatgaccaagaaccaggtgtccctgacctgcctggtcaagggcttctacccttccgacattgccgtggaatgggagtccaatggccagcctgagaacaactacaagaccacacctcctgtgctggactccgacggctccttctttctgtactctcgcctgaccgtggacaagtctagatggcaagagggcaacgtgttctcctgctctgtgctgcacgaggccctgcacaatcactacacccagaagtccctgtctctgtctcttggaggtggtggcggttctgcccctaccagctcctctaccaagaaaacccagctccagttggagcatctgctgctggacctccagatgattctgaacgggatcaacaactataagaaccccaagctgaccgccatgctgaccgctaagttcgccatgcccaagaaggccaccgagctgaagcacctccagtgcctggaagaagaactgaagcccctggaagaggtgctgaatctggcccagtccaagaacttccacctgaggccacgggacctgatcagcaacatcaacgtgatcgtgctggaactgaagggctccgagacaacctttatgtgcgagtacgccgacgagacagccaccatcgtggaatttctgaaccggtggatcaccttctgccagagcatcatctccacactgacc

SEQ ID NO: 26 - protein, 592 aa, Artificial Sequence
  fusion protein (GI102-M45)
VIHVTKEVKEVATLSCGHNVSVEELAQTRIYWQKEKKMVLTMMSGDMNIWPEYKNRTIFDITNNLSIVILALRPSDEGTYECVVLKYEKDAFKREHLAEVTLSVKADFPTPSISDFEIPTSNIRRIICSTSGGFPEPHLSWLENGEELNAINTTVSQDPETELYAVSSKLDFNMTTNHSFMCLIKYGHLRVNQTFNWNTTKQEHFPDNGSGGGGSGGGGSGGGGSAESKYGPPCPPCPAPEAAGGPSVFLFPPKPKDQLMISRTPEVTCVVVDVSQEDPEVQFNWYVDGVEVHNAKTKPREEQFNSTYRVVSVLTVLHQDWLNGKEYKCKVSNKGLPSSIEKTISKAKGQPREPQVYTLPPSQEEMTKNQVSLTCLVKGFYPSDIAVEWESNGQPENNYKTTPPVLDSDGSFFLYSRLTVDKSRWQEGNVFSCSVLHEALHNHYTQKSLSLSLGGGGGSAPTSSSTKKTQLQLEHLLLDLQMILNGINNYKNPKLTAMLTAKFAMPKKATELKHLQCLEEELKPLEEVLNLAQSKNFHLRPRDLISNINVIVLELKGSETTFMCEYADETATIVEFLNRWITFCQSIISTLT

SEQ ID NO: 27 - DNA, 1851 bp, Artificial Sequence
  nucleotiedes coding fusion protein (GI102-M61)
atggatgctatgctgagaggcctgtgttgcgtgctgctgctgtgtggcgctgtgttcgtgtctccttctcacgctgtgatccacgtgaccaaagaagtgaaagaggtcgccacactgtcctgcggccacaacgtttcagtggaagaactggcccagaccaggatctactggcagaaagaaaagaaaatggtgctgaccatgatgtccggcgacatgaacatctggcctgagtacaagaaccggaccatcttcgacatcaccaacaacctgtccatcgtgattctggccctgaggccttctgatgagggcacctatgagtgcgtggtgctgaagtacgagaaggacgccttcaagcgcgagcacctggctgaagtgacactgtccgtgaaggccgactttcccacaccttccatctccgacttcgagatccctacctccaacatccggcggatcatctgttctacctctggcggctttcctgagcctcacctgtcttggctggaaaacggcgaggaactgaacgccatcaacaccaccgtgtctcaggaccccgaaaccgagctgtacgctgtgtcctccaagctggacttcaacatgaccaccaaccacagcttcatgtgcctgattaagtacggccacctgagagtgaaccagaccttcaactggaacaccaccaagcaagagcacttccctgacaatggatctggcggcggaggttctggcggaggtggaagcggaggcggaggatctgctgagtctaagtatggccctccttgtcctccatgtcctgctccagaagctgctggcggaccctctgtgttcctgtttcctccaaagcctaaggaccagctcatgatctctcggacacccgaagtgacctgcgtggtggtggatgtgtctcaagaggaccctgaggtgcagttcaattggtacgtggacggcgtggaagtgcacaacgccaagaccaagcctagagaggaacagttcaactccacctacagagtggtgtccgtgctgaccgtgctgcaccaggattggctgaacggcaaagagtacaagtgcaaggtgtccaacaagggcctgccttccagcatcgaaaagaccatctccaaggctaagggccagcctagggaaccccaggtttacaccctgcctccaagccaagaggaaatgaccaagaaccaggtgtccctgacctgcctggtcaagggcttctacccttccgacattgccgtggaatgggagtccaatggccagcctgagaacaactacaagaccacacctcctgtgctggactccgacggctccttctttctgtactctcgcctgaccgtggacaagtctagatggcaagagggcaacgtgttctcctgctctgtgctgcacgaggccctgcacaatcactacacccagaagtccctgtctctgtctcttggaggtggtggcggttctgcccctaccagctcctctaccaagaaaacccagctccagttggagcatctgctgctggacctccagatgattctgaacgggatcaacaactataagaaccccaagctgaccgccatgctgaccgctaagttctacatgcccaagaaggccaccgagctgaagcacctccagtgcctggaaagggaactgaagcccctggaagaggtgctgaatctggcccagtccaagaacttccacctgaggccacgggacctgatcagcaacatcaacgtgatcgtgctggaactgaagggctccgagacaacctttatgtgcgagtacgccgacgagacagccaccatcgtggaatttctgaaccggtggatcaccttctgccagagcatcatctccacactgacc

SEQ ID NO: 28 - protein, 592 aa, Artificial Sequence
  fusion protein (GI102-M61)
VIHVTKEVKEVATLSCGHNVSVEELAQTRIYWQKEKKMVLTMMSGDMNIWPEYKNRTIFDITNNLSIVILALRPSDEGTYECVVLKYEKDAFKREHLAEVTLSVKADFPTPSISDFEIPTSNIRRIICSTSGGFPEPHLSWLENGEELNAINTTVSQDPETELYAVSSKLDFNMTTNHSFMCLIKYGHLRVNQTFNWNTTKQEHFPDNGSGGGGSGGGGSGGGGSAESKYGPPCPPCPAPEAAGGPSVFLFPPKPKDQLMISRTPEVTCVVVDVSQEDPEVQFNWYVDGVEVHNAKTKPREEQFNSTYRVVSVLTVLHQDWLNGKEYKCKVSNKGLPSSIEKTISKAKGQPREPQVYTLPPSQEEMTKNQVSLTCLVKGFYPSDIAVEWESNGQPENNYKTTPPVLDSDGSFFLYSRLTVDKSRWQEGNVFSCSVLHEALHNHYTQKSLSLSLGGGGGSAPTSSSTKKTQLQLEHLLLDLQMILNGINNYKNPKLTAMLTAKFYMPKKATELKHLQCLERELKPLEEVLNLAQSKNFHLRPRDLISNINVIVLELKGSETTFMCEYADETATIVEFLNRWITFCQSIISTLT

SEQ ID NO: 29 - DNA, 1857 bp, Artificial Sequence
  nucleotiedes coding fusion protein (GI102-M72)
atggatgctatgctgagaggcctgtgttgcgtgctgctgctgtgtggcgctgtgttcgtgtctccttctcacgctgtgatccacgtgaccaaagaagtgaaagaggtcgccacactgtcctgcggccacaacgtttcagtggaagaactggcccagaccaggatctactggcagaaagaaaagaaaatggtgctgaccatgatgtccggcgacatgaacatctggcctgagtacaagaaccggaccatcttcgacatcaccaacaacctgtccatcgtgattctggccctgaggccttctgatgagggcacctatgagtgcgtggtgctgaagtacgagaaggacgccttcaagcgcgagcacctggctgaagtgacactgtccgtgaaggccgactttcccacaccttccatctccgacttcgagatccctacctccaacatccggcggatcatctgttctacctctggcggctttcctgagcctcacctgtcttggctggaaaacggcgaggaactgaacgccatcaacaccaccgtgtctcaggaccccgaaaccgagctgtacgctgtgtcctccaagctggacttcaacatgaccaccaaccacagcttcatgtgcctgattaagtacggccacctgagagtgaaccagaccttcaactggaacaccaccaagcaagagcacttccctgacaatggatctggcggcggaggttctggcggaggtggaagcggaggcggaggatctgctgagtctaagtatggccctccttgtcctccatgtcctgctccagaagctgctggcggaccctctgtgttcctgtttcctccaaagcctaaggaccagctcatgatctctcggacacccgaagtgacctgcgtggtggtggatgtgtctcaagaggaccctgaggtgcagttcaattggtacgtggacggcgtggaagtgcacaacgccaagaccaagcctagagaggaacagttcaactccacctacagagtggtgtccgtgctgaccgtgctgcaccaggattggctgaacggcaaagagtacaagtgcaaggtgtccaacaagggcctgccttccagcatcgaaaagaccatctccaaggctaagggccagcctagggaaccccaggtttacaccctgcctccaagccaagaggaaatgaccaagaaccaggtgtccctgacctgcctggtcaagggcttctacccttccgacattgccgtggaatgggagtccaatggccagcctgagaacaactacaagaccacacctcctgtgctggactccgacggctccttctttctgtactctcgcctgaccgtggacaagtctagatggcaagagggcaacgtgttctcctgctctgtgctgcacgaggccctgcacaatcactacacccagaagtccctgtctctgtctcttggaggtggtggcggttctgcccctaccagctcctctaccaagaaaacccagctccagttggagcatctgctgctggacctccagatgattctgaacgggatcaacaactataagaaccccaagctgaccgccatgctgaccgctaagttctacatgcccaagaaggccaccgagctgaagcacctccagtgcctggaagaagaactgaagcccctggaagaggtgctgaatggggcccagtccaagaacttccacctgaggccacgggacctgatcagcaacatcaacgtgatcgtgctggaactgaagggctccgagacaacctttatgtgcgagtacgccgacgagacagccaccatcgtggaatttctgaaccggtggatcaccttctgccagagcatcatctccacactgacctgatga

SEQ ID NO: 30 - protein, 592 aa, Artificial Sequence
  fusion protein (GI102-M72)
VIHVTKEVKEVATLSCGHNVSVEELAQTRIYWQKEKKMVLTMMSGDMNIWPEYKNRTIFDITNNLSIVILALRPSDEGTYECVVLKYEKDAFKREHLAEVTLSVKADFPTPSISDFEIPTSNIRRIICSTSGGFPEPHLSWLENGEELNAINTTVSQDPETELYAVSSKLDFNMTTNHSFMCLIKYGHLRVNQTFNWNTTKQEHFPDNGSGGGGSGGGGSGGGGSAESKYGPPCPPCPAPEAAGGPSVFLFPPKPKDQLMISRTPEVTCVVVDVSQEDPEVQFNWYVDGVEVHNAKTKPREEQFNSTYRVVSVLTVLHQDWLNGKEYKCKVSNKGLPSSIEKTISKAKGQPREPQVYTLPPSQEEMTKNQVSLTCLVKGFYPSDIAVEWESNGQPENNYKTTPPVLDSDGSFFLYSRLTVDKSRWQEGNVFSCSVLHEALHNHYTQKSLSLSLGGGGGSAPTSSSTKKTQLQLEHLLLDLQMILNGINNYKNPKLTAMLTAKFYMPKKATELKHLQCLEEELKPLEEVLNGAQSKNFHLRPRDLISNINVIVLELKGSETTFMCEYADETATIVEFLNRWITFCQSIISTLT

SEQ ID NO: 31 - DNA, 1851 bp, Artificial Sequence
  nucleotiedes coding fusion protein (GI101w)
atggatgctatgctgagaggcctgtgttgcgtgctgctgctgtgtggcgctgtgttcgtgtctccttctcacgctgtgatccacgtgaccaaagaagtgaaagaggtcgccacactgtcctgcggccacaacgtttcagtggaagaactggcccagaccaggatctactggcagaaagaaaagaaaatggtgctgaccatgatgtccggcgacatgaacatctggcctgagtacaagaaccggaccatcttcgacatcaccaacaacctgtccatcgtgattctggccctgaggccttctgatgagggcacctatgagtgcgtggtgctgaagtacgagaaggacgccttcaagcgcgagcacctggctgaagtgacactgtccgtgaaggccgactttcccacaccttccatctccgacttcgagatccctacctccaacatccggcggatcatctgttctacctctggcggctttcctgagcctcacctgtcttggctggaaaacggcgaggaactgaacgccatcaacaccaccgtgtctcaggaccccgaaaccgagctgtacgctgtgtcctccaagctggacttcaacatgaccaccaaccacagcttcatgtgcctgattaagtacggccacctgagagtgaaccagaccttcaactggaacaccaccaagcaagagcacttccctgacaatggatctggcggcggaggttctggcggaggtggaagcggaggcggaggatctgctgagtctaagtatggccctccttgtcctccatgtcctgctccagaagctgctggcggaccctctgtgttcctgtttcctccaaagcctaaggaccagctcatgatctctcggacacccgaagtgacctgcgtggtggtggatgtgtctcaagaggaccctgaggtgcagttcaattggtacgtggacggcgtggaagtgcacaacgccaagaccaagcctagagaggaacagttcaactccacctacagagtggtgtccgtgctgaccgtgctgcaccaggattggctgaacggcaaagagtacaagtgcaaggtgtccaacaagggcctgccttccagcatcgaaaagaccatctccaaggctaagggccagcctagggaaccccaggtttacaccctgcctccaagccaagaggaaatgaccaagaaccaggtgtccctgacctgcctggtcaagggcttctacccttccgacattgccgtggaatgggagtccaatggccagcctgagaacaactacaagaccacacctcctgtgctggactccgacggctccttctttctgtactctcgcctgaccgtggacaagtctagatggcaagagggcaacgtgttctcctgctctgtgctgcacgaggccctgcacaatcactacacccagaagtccctgtctctgtctcttggaggtggtggcggttctgcccctaccagctcctctaccaagaaaacccagctccagttggagcatctgctgctggacctccagatgattctgaacgggatcaacaactataagaaccccaagctgacccgcatgctgacctttaagttctacatgcccaagaaggccaccgagctgaagcacctccagtgcctggaagaagaactgaagcccctggaagaggtgctgaatctggcccagtccaagaacttccacctgaggccacgggacctgatcagcaacatcaacgtgatcgtgctggaactgaagggctccgagacaacctttatgtgcgagtacgccgacgagacagccaccatcgtggaatttctgaaccggtggatcaccttctgccagagcatcatctccacactgacc

SEQ ID NO: 32 - protein, 592 aa, Artificial Sequence
  fusion protein (GI101w)
VIHVTKEVKEVATLSCGHNVSVEELAQTRIYWQKEKKMVLTMMSGDMNIWPEYKNRTIFDITNNLSIVILALRPSDEGTYECVVLKYEKDAFKREHLAEVTLSVKADFPTPSISDFEIPTSNIRRIICSTSGGFPEPHLSWLENGEELNAINTTVSQDPETELYAVSSKLDFNMTTNHSFMCLIKYGHLRVNQTFNWNTTKQEHFPDNGSGGGGSGGGGSGGGGSAESKYGPPCPPCPAPEAAGGPSVFLFPPKPKDQLMISRTPEVTCVVVDVSQEDPEVQFNWYVDGVEVHNAKTKPREEQFNSTYRVVSVLTVLHQDWLNGKEYKCKVSNKGLPSSIEKTISKAKGQPREPQVYTLPPSQEEMTKNQVSLTCLVKGFYPSDIAVEWESNGQPENNYKTTPPVLDSDGSFFLYSRLTVDKSRWQEGNVFSCSVLHEALHNHYTQKSLSLSLGGGGGSAPTSSSTKKTQLQLEHLLLDLQMILNGINNYKNPKLTRMLTFKFYMPKKATELKHLQCLEEELKPLEEVLNLAQSKNFHLRPRDLISNINVIVLELKGSETTFMCEYADETATIVEFLNRWITFCQSIISTLT

SEQ ID NO: 33 - DNA, 1848 bp, Artificial Sequence
  nucleotiedes coding fusion protein (mGI102-M61)
atggatgctatgctgagaggcctgtgttgcgtgctgctgctgtgtggcgctgtgttcgtgtctccttctcacgctgtggacgagcagctctccaagtccgtgaaggataaggtcctgctgccttgccggtacaactctcctcacgaggacgagtctgaggaccggatctactggcagaaacacgacaaggtggtgctgtccgtgatcgccggaaagctgaaagtgtggcctgagtacaagaacaggaccctgtacgacaacaccacctacagcctgatcatcctgggcctcgtgctgagcgatagaggcacctattcttgcgtggtgcagaagaaagagcggggcacctacgaagtgaagcacctggctctggtcaagctgtccatcaaggccgacttcagcacccctaacatcaccgagtctggcaacccttccgccgacaccaagagaatcacctgtttcgcctctggcggcttccctaagcctcggttctcttggctggaaaacggcagagagctgcccggcatcaataccaccatttctcaggacccagagtccgagctgtacaccatctccagccagctcgactttaacaccaccagaaaccacaccatcaagtgcctgattaagtacggcgacgcccacgtgtccgaggactttacttgggagaaacctcctgaggaccctcctgactctggatctggcggcggaggttctggcggaggtggaagcggaggcggaggatctgctgagtctaagtatggccctccttgtcctccatgtcctgctccagaagctgctggcggaccctctgtgttcctgtttcctccaaagcctaaggaccagctcatgatctctcggacccctgaagtgacctgcgtggtggtggatgtgtctcaagaggaccctgaggtgcagttcaattggtacgtggacggcgtggaagtgcacaacgccaagaccaagcctagagaggaacagttcaactccacctatagagtggtgtccgtgctgaccgtgctgcaccaggattggctgaacggcaaagagtacaagtgcaaggtgtccaacaagggcctgccttccagcatcgaaaagaccatcagcaaggctaagggccagcctagggaaccccaggtttacaccctgcctccaagccaagaggaaatgaccaagaaccaggtgtccctgacctgcctggtcaagggcttctacccttccgacattgccgtggaatgggagtccaatggccagcctgagaacaactacaagaccacacctcctgtgctggactccgacggctccttctttctgtactctcgcctgaccgtggacaagtctaggtggcaagagggcaacgtgttctcctgctctgtgctgcacgaggctctgcacaaccactacacccagaagtccctgtctctgtctcttggaggtggtggcggttctgcccctacctccagctctaccaagaaaacccagctccagttggagcatctgctgctggacctccagatgatcctgaatggcatcaacaattacaagaaccccaagctgaccgccatgctgaccgctaagttctacatgcccaagaaggccaccgagctgaagcacttgcagtgcctggaaagggaactgaagcccctggaagaagtgctgaatctggcccagtccaagaacttccacctgaggcctagggacctgatctccaacatcaacgtgatcgtgctggaactgaaaggctccgagacaaccttcatgtgcgagtacgccgacgagacagccaccatcgtggaatttctgaaccggtggatcaccttctgccagagcatcatctccacactgacc

SEQ ID NO: 34 - protein, 616 aa, Artificial Sequence
  fusion protein (mGI102-M61)
MDAMLRGLCCVLLLCGAVFVSPSHAVDEQLSKSVKDKVLLPCRYNSPHEDESEDRIYWQKHDKVVLSVIAGKLKVWPEYKNRTLYDNTTYSLIILGLVLSDRGTYSCVVQKKERGTYEVKHLALVKLSIKADFSTPNITESGNPSADTKRITCFASGGFPKPRFSWLENGRELPGINTTISQDPESELYTISSQLDFNTTRNHTIKCLIKYGDAHVSEDFTWEKPPEDPPDSGSGGGGSGGGGSGGGGSAESKYGPPCPPCPAPEAAGGPSVFLFPPKPKDQLMISRTPEVTCVVVDVSQEDPEVQFNWYVDGVEVHNAKTKPREEQFNSTYRVVSVLTVLHQDWLNGKEYKCKVSNKGLPSSIEKTISKAKGQPREPQVYTLPPSQEEMTKNQVSLTCLVKGFYPSDIAVEWESNGQPENNYKTTPPVLDSDGSFFLYSRLTVDKSRWQEGNVFSCSVLHEALHNHYTQKSLSLSLGGGGGSAPTSSSTKKTQLQLEHLLLDLQMILNGINNYKNPKLTAMLTAKFYMPKKATELKHLQCLERELKPLEEVLNLAQSKNFHLRPRDLISNINVIVLELKGSETTFMCEYADETATIVEFLNRWITFCQSIISTLT

SEQ ID NO: 35 - protein, 153 aa, Artificial Sequence
  wild type hIL-2
MYRMQLLSCIALSLALVTNSAPTSSSTKKTQLQLEHLLLDLQMILNGINNYKNPKLTRMLTFKFYMPKKATELKHLQCLEEELKPLEEVLNLAQSKNFHLRPRDLISNINVIVLELKGSETTFMCEYADETATIVEFLNRWITFCQSIISTLT

SEQ ID NO: 36 - protein, 158 aa, Artificial Sequence
  IL-2 with signal sequence
MDAMLRGLCCVLLLCGAVFVSPSHAAPTSSSTKKTQLQLEHLLLDLQMILNGINNYKNPKLTRMLTFKFYMPKKATELKHLQCLEEELKPLEEVLNLAQSKNFHLRPRDLISNINVIVLELKGSETTFMCEYADETATIVEFLNRWITFCQSIISTLT

SEQ ID NO: 37 - DNA, 474 bp, Artificial Sequence
  nucleotide sequence coding IL-2 with signal sequence
atggatgctatgctgagaggcctgtgttgcgtgctgctgctgtgtggcgctgtgttcgtgtctccttctcacgctgcccctaccagctcctctaccaagaaaacccagctccagttggagcatctgctgctggacctccagatgattctgaacgggatcaacaactataagaaccccaagctgacccgcatgctgacctttaagttctacatgcccaagaaggccaccgagctgaagcacctccagtgcctggaagaagaactgaagcccctggaagaggtgctgaatctggcccagtccaagaacttccacctgaggccacgggacctgatcagcaacatcaacgtgatcgtgctggaactgaagggctccgagacaacctttatgtgcgagtacgccgacgagacagccaccatcgtggaatttctgaaccggtggatcaccttctgccagagcatcatctccacactgacc

SEQ ID NO: 38 - protein, 222 aa, Artificial Sequence
  CD80 variant 1
MDAMLRGLCCVLLLCGAVFVSPSHAVIHVTKEVKEVATLSCGHNVSVEELAQTRIYWQKEKKMVLTMMSGDMNIWPEYKNRTIFDITNNLSIVILALRPSDEGTYECVVLKYEKDAFKREHLAEVTLSVKADFPTPSISDFEIPTSNIRRIICSTSGGFPEPHLSWLENGEELNAINTTVSQDPETELYAVSSKLDFNMTTNHSFMCLIKYGHLRVNQTFNW

SEQ ID NO: 39 - protein, 606 aa, Artificial Sequence
  GI-101-P1
MDAMLRGLCCVLLLCGAVFVSPSHAVIHVTKEVKEVATLSCGHNVSVEELAQTRIYWQKEKKMVLTMMSGDMNIWPEYKNRTIFDITNNLSIVILALRPSDEGTYECVVLKYEKDAFKREHLAEVTLSVKADFPTPSISDFEIPTSNIRRIICSTSGGFPEPHLSWLENGEELNAINTTVSQDPETELYAVSSKLDFNMTTNHSFMCLIKYGHLRVNQTFNWGSGGGGSGGGGSGGGGSAESKYGPPCPPCPAPEAAGGPSVFLFPPKPKDQLMISRTPEVTCVVVDVSQEDPEVQFNWYVDGVEVHNAKTKPREEQFNSTYRVVSVLTVLHQDWLNGKEYKCKVSNKGLPSSIEKTISKAKGQPREPQVYTLPPSQEEMTKNQVSLTCLVKGFYPSDIAVEWESNGQPENNYKTTPPVLDSDGSFFLYSRLTVDKSRWQEGNVFSCSVLHEALHNHYTQKSLSLSLGGGGGSAPTSSSTKKTQLQLEHLLLDLQMILNGINNYKNPKLTAMLTAKFYMPKKATELKHLQCLEEELKPLEEVLNLAQSKNFHLRPRDLISNINVIVLELKGSETTFMCEYADETATIVEFLNRWITFCQSIISTLT

SEQ ID NO: 40 - protein, 215 aa, Artificial Sequence
  CD80 variant 2
MDAMLRGLCCVLLLCGAVFVSPSHAVIHVTKEVKEVATLSCGHNVSVEELAQTRIYWQKEKKMVLTMMSGDMNIWPEYKNRTIFDITNNLSIVILALRPSDEGTYECVVLKYEKDAFKREHLAEVTLSVKADFPTPSISDFEIPTSNIRRIICSTSGGFPEPHLSWLENGEELNAINTTVSQDPETELYAVSSKLDFNMTTNHSFMCLIKYGHLR

SEQ ID NO: 41 - protein, 606 aa, Artificial Sequence; identical to SEQ ID NO: 39
  GI-101-P2

SEQ ID NO: 42 - protein, 210 aa, Artificial Sequence
  CD80 variant 3
MDAMLRGLCCVLLLCGAVFVSPSHAVIHVTKEVKEVATLSCGHNVSVEELAQTRIYWQKEKKMVLTMMSGDMNIWPEYKNRTIFDITNNLSIVILALRPSDEGTYECVVLKYEKDAFKREHLAEVTLSVKADFPTPSISDFEIPTSNIRRIICSTSGGFPEPHLSWLENGEELNAINTTVSQDPETELYAVSSKLDFNMTTNHSFMCLIK

SEQ ID NO: 43 - protein, 594 aa, Artificial Sequence
  GI-101-P3
MDAMLRGLCCVLLLCGAVFVSPSHAVIHVTKEVKEVATLSCGHNVSVEELAQTRIYWQKEKKMVLTMMSGDMNIWPEYKNRTIFDITNNLSIVILALRPSDEGTYECVVLKYEKDAFKREHLAEVTLSVKADFPTPSISDFEIPTSNIRRIICSTSGGFPEPHLSWLENGEELNAINTTVSQDPETELYAVSSKLDFNMTTNHSFMCLIKGSGGGGSGGGGSGGGGSAESKYGPPCPPCPAPEAAGGPSVFLFPPKPKDQLMISRTPEVTCVVVDVSQEDPEVQFNWYVDGVEVHNAKTKPREEQFNSTYRVVSVLTVLHQDWLNGKEYKCKVSNKGLPSSIEKTISKAKGQPREPQVYTLPPSQEEMTKNQVSLTCLVKGFYPSDIAVEWESNGQPENNYKTTPPVLDSDGSFFLYSRLTVDKSRWQEGNVFSCSVLHEALHNHYTQKSLSLSLGGGGGSAPTSSSTKKTQLQLEHLLLDLQMILNGINNYKNPKLTAMLTAKFYMPKKATELKHLQCLEEELKPLEEVLNLAQSKNFHLRPRDLISNINVIVLELKGSETTFMCEYADETATIVEFLNRWITFCQSIISTLT

SEQ ID NO: 44 - protein, 202 aa, Artificial Sequence
  CD80 variant 4
MDAMLRGLCCVLLLCGAVFVSPSHAVIHVTKEVKEVATLSCGHNVSVEELAQTRIYWQKEKKMVLTMMSGDMNIWPEYKNRTIFDITNNLSIVILALRPSDEGTYECVVLKYEKDAFKREHLAEVTLSVKADFPTPSISDFEIPTSNIRRIICSTSGGFPEPHLSWLENGEELNAINTTVSQDPETELYAVSSKLDFNMTTN

SEQ ID NO: 45 - protein, 586 aa, Artificial Sequence
  GI-101-P4
MDAMLRGLCCVLLLCGAVFVSPSHAVIHVTKEVKEVATLSCGHNVSVEELAQTRIYWQKEKKMVLTMMSGDMNIWPEYKNRTIFDITNNLSIVILALRPSDEGTYECVVLKYEKDAFKREHLAEVTLSVKADFPTPSISDFEIPTSNIRRIICSTSGGFPEPHLSWLENGEELNAINTTVSQDPETELYAVSSKLDFNMTTNGSGGGGSGGGGSGGGGSAESKYGPPCPPCPAPEAAGGPSVFLFPPKPKDQLMISRTPEVTCVVVDVSQEDPEVQFNWYVDGVEVHNAKTKPREEQFNSTYRVVSVLTVLHQDWLNGKEYKCKVSNKGLPSSIEKTISKAKGQPREPQVYTLPPSQEEMTKNQVSLTCLVKGFYPSDIAVEWESNGQPENNYKTTPPVLDSDGSFFLYSRLTVDKSRWQEGNVFSCSVLHEALHNHYTQKSLSLSLGGGGGSAPTSSSTKKTQLQLEHLLLDLQMILNGINNYKNPKLTAMLTAKFYMPKKATELKHLQCLEEELKPLEEVLNLAQSKNFHLRPRDLISNINVIVLELKGSETTFMCEYADETATIVEFLNRWITFCQSIISTLT

SEQ ID NO: 46 - protein, 199 aa, Artificial Sequence
  CD80 variant 5
MDAMLRGLCCVLLLCGAVFVSPSHAVIHVTKEVKEVATLSCGHNVSVEELAQTRIYWQKEKKMVLTMMSGDMNIWPEYKNRTIFDITNNLSIVILALRPSDEGTYECVVLKYEKDAFKREHLAEVTLSVKADFPTPSISDFEIPTSNIRRIICSTSGGFPEPHLSWLENGEELNAINTTVSQDPETELYAVSSKLDFNM

SEQ ID NO: 47 - protein, 583 aa, Artificial Sequence
  GI-101-P5
MDAMLRGLCCVLLLCGAVFVSPSHAVIHVTKEVKEVATLSCGHNVSVEELAQTRIYWQKEKKMVLTMMSGDMNIWPEYKNRTIFDITNNLSIVILALRPSDEGTYECVVLKYEKDAFKREHLAEVTLSVKADFPTPSISDFEIPTSNIRRIICSTSGGFPEPHLSWLENGEELNAINTTVSQDPETELYAVSSKLDFNMGSGGGGSGGGGSGGGGSAESKYGPPCPPCPAPEAAGGPSVFLFPPKPKDQLMISRTPEVTCVVVDVSQEDPEVQFNWYVDGVEVHNAKTKPREEQFNSTYRVVSVLTVLHQDWLNGKEYKCKVSNKGLPSSIEKTISKAKGQPREPQVYTLPPSQEEMTKNQVSLTCLVKGFYPSDIAVEWESNGQPENNYKTTPPVLDSDGSFFLYSRLTVDKSRWQEGNVFSCSVLHEALHNHYTQKSLSLSLGGGGGSAPTSSSTKKTQLQLEHLLLDLQMILNGINNYKNPKLTAMLTAKFYMPKKATELKHLQCLEEELKPLEEVLNLAQSKNFHLRPRDLISNINVIVLELKGSETTFMCEYADETATIVEFLNRWITFCQSIISTLT

SEQ ID NO: 48 - protein, 187 aa, Artificial Sequence
  CD80 variant 6
MDAMLRGLCCVLLLCGAVFVSPSHAVIHVTKEVKEVATLSCGHNVSVEELAQTRIYWQKEKKMVLTMMSGDMNIWPEYKNRTIFDITNNLSIVILALRPSDEGTYECVVLKYEKDAFKREHLAEVTLSVKADFPTPSISDFEIPTSNIRRIICSTSGGFPEPHLSWLENGEELNAINTTVSQDPETE

SEQ ID NO: 49 - protein, 571 aa, Artificial Sequence
  GI-101-P6
MDAMLRGLCCVLLLCGAVFVSPSHAVIHVTKEVKEVATLSCGHNVSVEELAQTRIYWQKEKKMVLTMMSGDMNIWPEYKNRTIFDITNNLSIVILALRPSDEGTYECVVLKYEKDAFKREHLAEVTLSVKADFPTPSISDFEIPTSNIRRIICSTSGGFPEPHLSWLENGEELNAINTTVSQDPETEGSGGGGSGGGGSGGGGSAESKYGPPCPPCPAPEAAGGPSVFLFPPKPKDQLMISRTPEVTCVVVDVSQEDPEVQFNWYVDGVEVHNAKTKPREEQFNSTYRVVSVLTVLHQDWLNGKEYKCKVSNKGLPSSIEKTISKAKGQPREPQVYTLPPSQEEMTKNQVSLTCLVKGFYPSDIAVEWESNGQPENNYKTTPPVLDSDGSFFLYSRLTVDKSRWQEGNVFSCSVLHEALHNHYTQKSLSLSLGGGGGSAPTSSSTKKTQLQLEHLLLDLQMILNGINNYKNPKLTAMLTAKFYMPKKATELKHLQCLEEELKPLEEVLNLAQSKNFHLRPRDLISNINVIVLELKGSETTFMCEYADETATIVEFLNRWITFCQSIISTLT

SEQ ID NO: 50 - protein, 183 aa, Artificial Sequence
  CD80 variant 7
MDAMLRGLCCVLLLCGAVFVSPSHAVIHVTKEVKEVATLSCGHNVSVEELAQTRIYWQKEKKMVLTMMSGDMNIWPEYKNRTIFDITNNLSIVILALRPSDEGTYECVVLKYEKDAFKREHLAEVTLSVKADFPTPSISDFEIPTSNIRRIICSTSGGFPEPHLSWLENGEELNAINTTVSQD

SEQ ID NO: 51 - protein, 567 aa, Artificial Sequence
  GI-101-P7
MDAMLRGLCCVLLLCGAVFVSPSHAVIHVTKEVKEVATLSCGHNVSVEELAQTRIYWQKEKKMVLTMMSGDMNIWPEYKNRTIFDITNNLSIVILALRPSDEGTYECVVLKYEKDAFKREHLAEVTLSVKADFPTPSISDFEIPTSNIRRIICSTSGGFPEPHLSWLENGEELNAINTTVSQDGSGGGGSGGGGSGGGGSAESKYGPPCPPCPAPEAAGGPSVFLFPPKPKDQLMISRTPEVTCVVVDVSQEDPEVQFNWYVDGVEVHNAKTKPREEQFNSTYRVVSVLTVLHQDWLNGKEYKCKVSNKGLPSSIEKTISKAKGQPREPQVYTLPPSQEEMTKNQVSLTCLVKGFYPSDIAVEWESNGQPENNYKTTPPVLDSDGSFFLYSRLTVDKSRWQEGNVFSCSVLHEALHNHYTQKSLSLSLGGGGGSAPTSSSTKKTQLQLEHLLLDLQMILNGINNYKNPKLTAMLTAKFYMPKKATELKHLQCLEEELKPLEEVLNLAQSKNFHLRPRDLISNINVIVLELKGSETTFMCEYADETATIVEFLNRWITFCQSIISTLT

SEQ ID NO: 52 - protein, 175 aa, Artificial Sequence
  CD80 variant 8
MDAMLRGLCCVLLLCGAVFVSPSHAVIHVTKEVKEVATLSCGHNVSVEELAQTRIYWQKEKKMVLTMMSGDMNIWPEYKNRTIFDITNNLSIVILALRPSDEGTYECVVLKYEKDAFKREHLAEVTLSVKADFPTPSISDFEIPTSNIRRIICSTSGGFPEPHLSWLENGEELNA

SEQ ID NO: 53 - protein, 559 aa, Artificial Sequence
  GI-101-P8
MDAMLRGLCCVLLLCGAVFVSPSHAVIHVTKEVKEVATLSCGHNVSVEELAQTRIYWQKEKKMVLTMMSGDMNIWPEYKNRTIFDITNNLSIVILALRPSDEGTYECVVLKYEKDAFKREHLAEVTLSVKADFPTPSISDFEIPTSNIRRIICSTSGGFPEPHLSWLENGEELNAGSGGGGSGGGGSGGGGSAESKYGPPCPPCPAPEAAGGPSVFLFPPKPKDQLMISRTPEVTCVVVDVSQEDPEVQFNWYVDGVEVHNAKTKPREEQFNSTYRVVSVLTVLHQDWLNGKEYKCKVSNKGLPSSIEKTISKAKGQPREPQVYTLPPSQEEMTKNQVSLTCLVKGFYPSDIAVEWESNGQPENNYKTTPPVLDSDGSFFLYSRLTVDKSRWQEGNVFSCSVLHEALHNHYTQKSLSLSLGGGGGSAPTSSSTKKTQLQLEHLLLDLQMILNGINNYKNPKLTAMLTAKFYMPKKATELKHLQCLEEELKPLEEVLNLAQSKNFHLRPRDLISNINVIVLELKGSETTFMCEYADETATIVEFLNRWITFCQSIISTLT

SEQ ID NO: 54 - protein, 136 aa, Artificial Sequence
  CD80 variant 9
MDAMLRGLCCVLLLCGAVFVSPSHAVIHVTKEVKEVATLSCGHNVSVEELAQTRIYWQKEKKMVLTMMSGDMNIWPEYKNRTIFDITNNLSIVILALRPSDEGTYECVVLKYEKDAFKREHLAEVTLSVKADFPTP

SEQ ID NO: 55 - protein, 520 aa, Artificial Sequence
  GI-101-P9
MDAMLRGLCCVLLLCGAVFVSPSHAVIHVTKEVKEVATLSCGHNVSVEELAQTRIYWQKEKKMVLTMMSGDMNIWPEYKNRTIFDITNNLSIVILALRPSDEGTYECVVLKYEKDAFKREHLAEVTLSVKADFPTPGSGGGGSGGGGSGGGGSAESKYGPPCPPCPAPEAAGGPSVFLFPPKPKDQLMISRTPEVTCVVVDVSQEDPEVQFNWYVDGVEVHNAKTKPREEQFNSTYRVVSVLTVLHQDWLNGKEYKCKVSNKGLPSSIEKTISKAKGQPREPQVYTLPPSQEEMTKNQVSLTCLVKGFYPSDIAVEWESNGQPENNYKTTPPVLDSDGSFFLYSRLTVDKSRWQEGNVFSCSVLHEALHNHYTQKSLSLSLGGGGGSAPTSSSTKKTQLQLEHLLLDLQMILNGINNYKNPKLTAMLTAKFYMPKKATELKHLQCLEEELKPLEEVLNLAQSKNFHLRPRDLISNINVIVLELKGSETTFMCEYADETATIVEFLNRWITFCQSIISTLT

SEQ ID NO: 56 - protein, 130 aa, Artificial Sequence
  CD80 variant 10
MDAMLRGLCCVLLLCGAVFVSPSHAEVKEVATLSCGHNVSVEELAQTRIYWQKEKKMVLTMMSGDMNIWPEYKNRTIFDITNNLSIVILALRPSDEGTYECVVLKYEKDAFKREHLAEVTLSVKADFPTP

SEQ ID NO: 57 - protein, 514 aa, Artificial Sequence
  GI-101-P10
MDAMLRGLCCVLLLCGAVFVSPSHAEVKEVATLSCGHNVSVEELAQTRIYWQKEKKMVLTMMSGDMNIWPEYKNRTIFDITNNLSIVILALRPSDEGTYECVVLKYEKDAFKREHLAEVTLSVKADFPTPGSGGGGSGGGGSGGGGSAESKYGPPCPPCPAPEAAGGPSVFLFPPKPKDQLMISRTPEVTCVVVDVSQEDPEVQFNWYVDGVEVHNAKTKPREEQFNSTYRVVSVLTVLHQDWLNGKEYKCKVSNKGLPSSIEKTISKAKGQPREPQVYTLPPSQEEMTKNQVSLTCLVKGFYPSDIAVEWESNGQPENNYKTTPPVLDSDGSFFLYSRLTVDKSRWQEGNVFSCSVLHEALHNHYTQKSLSLSLGGGGGSAPTSSSTKKTQLQLEHLLLDLQMILNGINNYKNPKLTAMLTAKFYMPKKATELKHLQCLEEELKPLEEVLNLAQSKNFHLRPRDLISNINVIVLELKGSETTFMCEYADETATIVEFLNRWITFCQSIISTLT

SEQ ID NO: 58 - protein, 125 aa, Artificial Sequence
  CD80 variant 11
MDAMLRGLCCVLLLCGAVFVSPSHAATLSCGHNVSVEELAQTRIYWQKEKKMVLTMMSGDMNIWPEYKNRTIFDITNNLSIVILALRPSDEGTYECVVLKYEKDAFKREHLAEVTLSVKADFPTP

SEQ ID NO: 59 - protein, 509 aa, Artificial Sequence
  GI-101-P11
MDAMLRGLCCVLLLCGAVFVSPSHAATLSCGHNVSVEELAQTRIYWQKEKKMVLTMMSGDMNIWPEYKNRTIFDITNNLSIVILALRPSDEGTYECVVLKYEKDAFKREHLAEVTLSVKADFPTPGSGGGGSGGGGSGGGGSAESKYGPPCPPCPAPEAAGGPSVFLFPPKPKDQLMISRTPEVTCVVVDVSQEDPEVQFNWYVDGVEVHNAKTKPREEQFNSTYRVVSVLTVLHQDWLNGKEYKCKVSNKGLPSSIEKTISKAKGQPREPQVYTLPPSQEEMTKNQVSLTCLVKGFYPSDIAVEWESNGQPENNYKTTPPVLDSDGSFFLYSRLTVDKSRWQEGNVFSCSVLHEALHNHYTQKSLSLSLGGGGGSAPTSSSTKKTQLQLEHLLLDLQMILNGINNYKNPKLTAMLTAKFYMPKKATELKHLQCLEEELKPLEEVLNLAQSKNFHLRPRDLISNINVIVLELKGSETTFMCEYADETATIVEFLNRWITFCQSIISTLT

SEQ ID NO: 60 - protein, 116 aa, Artificial Sequence
  CD80 variant 12
MDAMLRGLCCVLLLCGAVFVSPSHASVEELAQTRIYWQKEKKMVLTMMSGDMNIWPEYKNRTIFDITNNLSIVILALRPSDEGTYECVVLKYEKDAFKREHLAEVTLSVKADFPTP

SEQ ID NO: 61 - protein, 500 aa, Artificial Sequence
  GI-101-P12
MDAMLRGLCCVLLLCGAVFVSPSHASVEELAQTRIYWQKEKKMVLTMMSGDMNIWPEYKNRTIFDITNNLSIVILALRPSDEGTYECVVLKYEKDAFKREHLAEVTLSVKADFPTPGSGGGGSGGGGSGGGGSAESKYGPPCPPCPAPEAAGGPSVFLFPPKPKDQLMISRTPEVTCVVVDVSQEDPEVQFNWYVDGVEVHNAKTKPREEQFNSTYRVVSVLTVLHQDWLNGKEYKCKVSNKGLPSSIEKTISKAKGQPREPQVYTLPPSQEEMTKNQVSLTCLVKGFYPSDIAVEWESNGQPENNYKTTPPVLDSDGSFFLYSRLTVDKSRWQEGNVFSCSVLHEALHNHYTQKSLSLSLGGGGGSAPTSSSTKKTQLQLEHLLLDLQMILNGINNYKNPKLTAMLTAKFYMPKKATELKHLQCLEEELKPLEEVLNLAQSKNFHLRPRDLISNINVIVLELKGSETTFMCEYADETATIVEFLNRWITFCQSIISTLT

SEQ ID NO: 62 - protein, 110 aa, Artificial Sequence
  CD80 variant 13
MDAMLRGLCCVLLLCGAVFVSPSHAQTRIYWQKEKKMVLTMMSGDMNIWPEYKNRTIFDITNNLSIVILALRPSDEGTYECVVLKYEKDAFKREHLAEVTLSVKADFPTP

SEQ ID NO: 63 - protein, 494 aa, Artificial Sequence
  GI-101-P13
MDAMLRGLCCVLLLCGAVFVSPSHAQTRIYWQKEKKMVLTMMSGDMNIWPEYKNRTIFDITNNLSIVILALRPSDEGTYECVVLKYEKDAFKREHLAEVTLSVKADFPTPGSGGGGSGGGGSGGGGSAESKYGPPCPPCPAPEAAGGPSVFLFPPKPKDQLMISRTPEVTCVVVDVSQEDPEVQFNWYVDGVEVHNAKTKPREEQFNSTYRVVSVLTVLHQDWLNGKEYKCKVSNKGLPSSIEKTISKAKGQPREPQVYTLPPSQEEMTKNQVSLTCLVKGFYPSDIAVEWESNGQPENNYKTTPPVLDSDGSFFLYSRLTVDKSRWQEGNVFSCSVLHEALHNHYTQKSLSLSLGGGGGSAPTSSSTKKTQLQLEHLLLDLQMILNGINNYKNPKLTAMLTAKFYMPKKATELKHLQCLEEELKPLEEVLNLAQSKNFHLRPRDLISNINVIVLELKGSETTFMCEYADETATIVEFLNRWITFCQSIISTLT

SEQ ID NO: 64 - protein, 103 aa, Artificial Sequence
  CD80 variant 14
MDAMLRGLCCVLLLCGAVFVSPSHAQTRIYWQKEKKMVLTMMSGDMNIWPEYKNRTIFDITNNLSIVILALRPSDEGTYECVVLKYEKDAFKREHLAEVTLSV

SEQ ID NO: 65 - protein, 487 aa, Artificial Sequence
  GI-101-P14
MDAMLRGLCCVLLLCGAVFVSPSHAQTRIYWQKEKKMVLTMMSGDMNIWPEYKNRTIFDITNNLSIVILALRPSDEGTYECVVLKYEKDAFKREHLAEVTLSVGSGGGGSGGGGSGGGGSAESKYGPPCPPCPAPEAAGGPSVFLFPPKPKDQLMISRTPEVTCVVVDVSQEDPEVQFNWYVDGVEVHNAKTKPREEQFNSTYRVVSVLTVLHQDWLNGKEYKCKVSNKGLPSSIEKTISKAKGQPREPQVYTLPPSQEEMTKNQVSLTCLVKGFYPSDIAVEWESNGQPENNYKTTPPVLDSDGSFFLYSRLTVDKSRWQEGNVFSCSVLHEALHNHYTQKSLSLSLGGGGGSAPTSSSTKKTQLQLEHLLLDLQMILNGINNYKNPKLTAMLTAKFYMPKKATELKHLQCLEEELKPLEEVLNLAQSKNFHLRPRDLISNINVIVLELKGSETTFMCEYADETATIVEFLNRWITFCQSIISTLT

SEQ ID NO: 66 - protein, 93 aa, Artificial Sequence
  CD80 variant 15
MDAMLRGLCCVLLLCGAVFVSPSHASGDMNIWPEYKNRTIFDITNNLSIVILALRPSDEGTYECVVLKYEKDAFKREHLAEVTLSVKADFPTP

SEQ ID NO: 67 - protein, 477 aa, Artificial Sequence
  GI-101-P15
MDAMLRGLCCVLLLCGAVFVSPSHASGDMNIWPEYKNRTIFDITNNLSIVILALRPSDEGTYECVVLKYEKDAFKREHLAEVTLSVKADFPTPGSGGGGSGGGGSGGGGSAESKYGPPCPPCPAPEAAGGPSVFLFPPKPKDQLMISRTPEVTCVVVDVSQEDPEVQFNWYVDGVEVHNAKTKPREEQFNSTYRVVSVLTVLHQDWLNGKEYKCKVSNKGLPSSIEKTISKAKGQPREPQVYTLPPSQEEMTKNQVSLTCLVKGFYPSDIAVEWESNGQPENNYKTTPPVLDSDGSFFLYSRLTVDKSRWQEGNVFSCSVLHEALHNHYTQKSLSLSLGGGGGSAPTSSSTKKTQLQLEHLLLDLQMILNGINNYKNPKLTAMLTAKFYMPKKATELKHLQCLEEELKPLEEVLNLAQSKNFHLRPRDLISNINVIVLELKGSETTFMCEYADETATIVEFLNRWITFCQSIISTLT

SEQ ID NO: 68 - protein, 49 aa, Artificial Sequence
  CD80 variant 16
MDAMLRGLCCVLLLCGAVFVSPSHAQTRIYWQKEKKMVLTMMSGDMNIW

SEQ ID NO: 69 - protein, 433 aa, Artificial Sequence
  GI-101-P16
MDAMLRGLCCVLLLCGAVFVSPSHAQTRIYWQKEKKMVLTMMSGDMNIWGSGGGGSGGGGSGGGGSAESKYGPPCPPCPAPEAAGGPSVFLFPPKPKDQLMISRTPEVTCVVVDVSQEDPEVQFNWYVDGVEVHNAKTKPREEQFNSTYRVVSVLTVLHQDWLNGKEYKCKVSNKGLPSSIEKTISKAKGQPREPQVYTLPPSQEEMTKNQVSLTCLVKGFYPSDIAVEWESNGQPENNYKTTPPVLDSDGSFFLYSRLTVDKSRWQEGNVFSCSVLHEALHNHYTQKSLSLSLGGGGGSAPTSSSTKKTQLQLEHLLLDLQMILNGINNYKNPKLTAMLTAKFYMPKKATELKHLQCLEEELKPLEEVLNLAQSKNFHLRPRDLISNINVIVLELKGSETTFMCEYADETATIVEFLNRWITFCQSIISTLT

SEQ ID NO: 70 - protein, 42 aa, Artificial Sequence
  CD80 variant 17
MDAMLRGLCCVLLLCGAVFVSPSHAQTRIYWQKEKKMVLTMM

SEQ ID NO: 71 - protein, 426 aa, Artificial Sequence
  GI-101-P17
MDAMLRGLCCVLLLCGAVFVSPSHAQTRIYWQKEKKMVLTMMGSGGGGSGGGGSGGGGSAESKYGPPCPPCPAPEAAGGPSVFLFPPKPKDQLMISRTPEVTCVVVDVSQEDPEVQFNWYVDGVEVHNAKTKPREEQFNSTYRVVSVLTVLHQDWLNGKEYKCKVSNKGLPSSIEKTISKAKGQPREPQVYTLPPSQEEMTKNQVSLTCLVKGFYPSDIAVEWESNGQPENNYKTTPPVLDSDGSFFLYSRLTVDKSRWQEGNVFSCSVLHEALHNHYTQKSLSLSLGGGGGSAPTSSSTKKTQLQLEHLLLDLQMILNGINNYKNPKLTAMLTAKFYMPKKATELKHLQCLEEELKPLEEVLNLAQSKNFHLRPRDLISNINVIVLELKGSETTFMCEYADETATIVEFLNRWITFCQSIISTLT

SEQ ID NO: 72 - protein, 52 aa, Artificial Sequence
  CD80 variant 18
MDAMLRGLCCVLLLCGAVFVSPSHAGTYECVVLKYEKDAFKREHLAEVTLSV

SEQ ID NO: 73 - protein, 436 aa, Artificial Sequence
  GI-101-P18
MDAMLRGLCCVLLLCGAVFVSPSHAGTYECVVLKYEKDAFKREHLAEVTLSVGSGGGGSGGGGSGGGGSAESKYGPPCPPCPAPEAAGGPSVFLFPPKPKDQLMISRTPEVTCVVVDVSQEDPEVQFNWYVDGVEVHNAKTKPREEQFNSTYRVVSVLTVLHQDWLNGKEYKCKVSNKGLPSSIEKTISKAKGQPREPQVYTLPPSQEEMTKNQVSLTCLVKGFYPSDIAVEWESNGQPENNYKTTPPVLDSDGSFFLYSRLTVDKSRWQEGNVFSCSVLHEALHNHYTQKSLSLSLGGGGGSAPTSSSTKKTQLQLEHLLLDLQMILNGINNYKNPKLTAMLTAKFYMPKKATELKHLQCLEEELKPLEEVLNLAQSKNFHLRPRDLISNINVIVLELKGSETTFMCEYADETATIVEFLNRWITFCQSIISTLT

SEQ ID NO: 74 - protein, 233 aa, Artificial Sequence
  GI-101-CD80
MDAMLRGLCCVLLLCGAVFVSPSHAVIHVTKEVKEVATLSCGHNVSVEELAQTRIYWQKEKKMVLTMMSGDMNIWPEYKNRTIFDITNNLSIVILALRPSDEGTYECVVLKYEKDAFKREHLAEVTLSVKADFPTPSISDFEIPTSNIRRIICSTSGGFPEPHLSWLENGEELNAINTTVSQDPETELYAVSSKLDFNMTTNHSFMCLIKYGHLRVNQTFNWNTTKQEHFPDN

SEQ ID NO: 75 - protein, 612 aa, Artificial Sequence
  GI-101-P19
MDAMLRGLCCVLLLCGAVFVSPSHAVIHVTKEVKEVATLSCGHNVSVEELAQTRIYWQKEKKMVLTMMSGDMNIWPEYKNRTIFDITNNLSIVILALRPSDEGTYECVVLKYEKDAFKREHLAEVTLSVKADFPTPSISDFEIPTSNIRRIICSTSGGFPEPHLSWLENGEELNAINTTVSQDPETELYAVSSKLDFNMTTNHSFMCLIKYGHLRVNQTFNWNTTKQEHFPDNGSGGGGSGGGGSGGGGSAESKYGPPCPPCPAPEAAGGPSVFLFPPKPKDQLMISRTPEVTCVVVDVSQEDPEVQFNWYVDGVEVHNAKTKPREEQFNSTYRVVSVLTVLHQDWLNGKEYKCKVSNKGLPSSIEKTISKAKGQPREPQVYTLPPSQEEMTKNQVSLTCLVKGFYPSDIAVEWESNGQPENNYKTTPPVLDSDGSFFLYSRLTVDKSRWQEGNVFSCSVLHEALHNHYTQKSLSLSLGAPTSSSTKKTQLQLEHLLLDLQMILNGINNYKNPKLTAMLTAKFYMPKKATELKHLQCLEEELKPLEEVLNLAQSKNFHLRPRDLISNINVIVLELKGSETTFMCEYADETATIVEFLNRWITFCQSIISTLT

SEQ ID NO: 76 - protein, 5 aa, Artificial Sequence
  Linker2 variant 20
EAAAK

SEQ ID NO: 77 - protein, 617 aa, Artificial Sequence
  GI-101-P20
MDAMLRGLCCVLLLCGAVFVSPSHAVIHVTKEVKEVATLSCGHNVSVEELAQTRIYWQKEKKMVLTMMSGDMNIWPEYKNRTIFDITNNLSIVILALRPSDEGTYECVVLKYEKDAFKREHLAEVTLSVKADFPTPSISDFEIPTSNIRRIICSTSGGFPEPHLSWLENGEELNAINTTVSQDPETELYAVSSKLDFNMTTNHSFMCLIKYGHLRVNQTFNWNTTKQEHFPDNGSGGGGSGGGGSGGGGSAESKYGPPCPPCPAPEAAGGPSVFLFPPKPKDQLMISRTPEVTCVVVDVSQEDPEVQFNWYVDGVEVHNAKTKPREEQFNSTYRVVSVLTVLHQDWLNGKEYKCKVSNKGLPSSIEKTISKAKGQPREPQVYTLPPSQEEMTKNQVSLTCLVKGFYPSDIAVEWESNGQPENNYKTTPPVLDSDGSFFLYSRLTVDKSRWQEGNVFSCSVLHEALHNHYTQKSLSLSLGEAAAKAPTSSSTKKTQLQLEHLLLDLQMILNGINNYKNPKLTAMLTAKFYMPKKATELKHLQCLEEELKPLEEVLNLAQSKNFHLRPRDLISNINVIVLELKGSETTFMCEYADETATIVEFLNRWITFCQSIISTLT

SEQ ID NO: 78 - protein, 10 aa, Artificial Sequence
  Linker2 variant 21
EAAAKEAAAK

SEQ ID NO: 79 - protein, 622 aa, Artificial Sequence
  GI-101-P21
MDAMLRGLCCVLLLCGAVFVSPSHAVIHVTKEVKEVATLSCGHNVSVEELAQTRIYWQKEKKMVLTMMSGDMNIWPEYKNRTIFDITNNLSIVILALRPSDEGTYECVVLKYEKDAFKREHLAEVTLSVKADFPTPSISDFEIPTSNIRRIICSTSGGFPEPHLSWLENGEELNAINTTVSQDPETELYAVSSKLDFNMTTNHSFMCLIKYGHLRVNQTFNWNTTKQEHFPDNGSGGGGSGGGGSGGGGSAESKYGPPCPPCPAPEAAGGPSVFLFPPKPKDQLMISRTPEVTCVVVDVSQEDPEVQFNWYVDGVEVHNAKTKPREEQFNSTYRVVSVLTVLHQDWLNGKEYKCKVSNKGLPSSIEKTISKAKGQPREPQVYTLPPSQEEMTKNQVSLTCLVKGFYPSDIAVEWESNGQPENNYKTTPPVLDSDGSFFLYSRLTVDKSRWQEGNVFSCSVLHEALHNHYTQKSLSLSLGEAAAKEAAAKAPTSSSTKKTQLQLEHLLLDLQMILNGINNYKNPKLTAMLTAKFYMPKKATELKHLQCLEEELKPLEEVLNLAQSKNFHLRPRDLISNINVIVLELKGSETTFMCEYADETATIVEFLNRWITFCQSIISTLT

SEQ ID NO: 80 - protein, 20 aa, Artificial Sequence
  Linker2 variant 22
EAAAKEAAAKEAAAKEAAAK

SEQ ID NO: 81 - protein, 632 aa, Artificial Sequence
  GI-101-P22
MDAMLRGLCCVLLLCGAVFVSPSHAVIHVTKEVKEVATLSCGHNVSVEELAQTRIYWQKEKKMVLTMMSGDMNIWPEYKNRTIFDITNNLSIVILALRPSDEGTYECVVLKYEKDAFKREHLAEVTLSVKADFPTPSISDFEIPTSNIRRIICSTSGGFPEPHLSWLENGEELNAINTTVSQDPETELYAVSSKLDFNMTTNHSFMCLIKYGHLRVNQTFNWNTTKQEHFPDNGSGGGGSGGGGSGGGGSAESKYGPPCPPCPAPEAAGGPSVFLFPPKPKDQLMISRTPEVTCVVVDVSQEDPEVQFNWYVDGVEVHNAKTKPREEQFNSTYRVVSVLTVLHQDWLNGKEYKCKVSNKGLPSSIEKTISKAKGQPREPQVYTLPPSQEEMTKNQVSLTCLVKGFYPSDIAVEWESNGQPENNYKTTPPVLDSDGSFFLYSRLTVDKSRWQEGNVFSCSVLHEALHNHYTQKSLSLSLGEAAAKEAAAKEAAAKEAAAKAPTSSSTKKTQLQLEHLLLDLQMILNGINNYKNPKLTAMLTAKFYMPKKATELKHLQCLEEELKPLEEVLNLAQSKNFHLRPRDLISNINVIVLELKGSETTFMCEYADETATIVEFLNRWITFCQSIISTLT

SEQ ID NO: 82 - protein, 10 aa, Artificial Sequence
  Linker2 variant 23
GGGGSGGGGS

SEQ ID NO: 83 - protein, 622 aa, Artificial Sequence
  GI-101-P23
MDAMLRGLCCVLLLCGAVFVSPSHAVIHVTKEVKEVATLSCGHNVSVEELAQTRIYWQKEKKMVLTMMSGDMNIWPEYKNRTIFDITNNLSIVILALRPSDEGTYECVVLKYEKDAFKREHLAEVTLSVKADFPTPSISDFEIPTSNIRRIICSTSGGFPEPHLSWLENGEELNAINTTVSQDPETELYAVSSKLDFNMTTNHSFMCLIKYGHLRVNQTFNWNTTKQEHFPDNGSGGGGSGGGGSGGGGSAESKYGPPCPPCPAPEAAGGPSVFLFPPKPKDQLMISRTPEVTCVVVDVSQEDPEVQFNWYVDGVEVHNAKTKPREEQFNSTYRVVSVLTVLHQDWLNGKEYKCKVSNKGLPSSIEKTISKAKGQPREPQVYTLPPSQEEMTKNQVSLTCLVKGFYPSDIAVEWESNGQPENNYKTTPPVLDSDGSFFLYSRLTVDKSRWQEGNVFSCSVLHEALHNHYTQKSLSLSLGGGGGSGGGGSAPTSSSTKKTQLQLEHLLLDLQMILNGINNYKNPKLTAMLTAKFYMPKKATELKHLQCLEEELKPLEEVLNLAQSKNFHLRPRDLISNINVIVLELKGSETTFMCEYADETATIVEFLNRWITFCQSIISTLT

SEQ ID NO: 84 - protein, 20 aa, Artificial Sequence
  Linker2 variant 24
GGGGSGGGGSGGGGSGGGGS

SEQ ID NO: 85 - protein, 632 aa, Artificial Sequence
  GI-101-P24
MDAMLRGLCCVLLLCGAVFVSPSHAVIHVTKEVKEVATLSCGHNVSVEELAQTRIYWQKEKKMVLTMMSGDMNIWPEYKNRTIFDITNNLSIVILALRPSDEGTYECVVLKYEKDAFKREHLAEVTLSVKADFPTPSISDFEIPTSNIRRIICSTSGGFPEPHLSWLENGEELNAINTTVSQDPETELYAVSSKLDFNMTTNHSFMCLIKYGHLRVNQTFNWNTTKQEHFPDNGSGGGGSGGGGSGGGGSAESKYGPPCPPCPAPEAAGGPSVFLFPPKPKDQLMISRTPEVTCVVVDVSQEDPEVQFNWYVDGVEVHNAKTKPREEQFNSTYRVVSVLTVLHQDWLNGKEYKCKVSNKGLPSSIEKTISKAKGQPREPQVYTLPPSQEEMTKNQVSLTCLVKGFYPSDIAVEWESNGQPENNYKTTPPVLDSDGSFFLYSRLTVDKSRWQEGNVFSCSVLHEALHNHYTQKSLSLSLGGGGGSGGGGSGGGGSGGGGSAPTSSSTKKTQLQLEHLLLDLQMILNGINNYKNPKLTAMLTAKFYMPKKATELKHLQCLEEELKPLEEVLNLAQSKNFHLRPRDLISNINVIVLELKGSETTFMCEYADETATIVEFLNRWITFCQSIISTLT

SEQ ID NO: 86 - protein, 13 aa, Artificial Sequence
  Linker1 variant 25
AESKYGPPCPPCP

SEQ ID NO: 87 - protein, 600 aa, Artificial Sequence
  GI-101-P25
MDAMLRGLCCVLLLCGAVFVSPSHAVIHVTKEVKEVATLSCGHNVSVEELAQTRIYWQKEKKMVLTMMSGDMNIWPEYKNRTIFDITNNLSIVILALRPSDEGTYECVVLKYEKDAFKREHLAEVTLSVKADFPTPSISDFEIPTSNIRRIICSTSGGFPEPHLSWLENGEELNAINTTVSQDPETELYAVSSKLDFNMTTNHSFMCLIKYGHLRVNQTFNWNTTKQEHFPDNAESKYGPPCPPCPAPEAAGGPSVFLFPPKPKDQLMISRTPEVTCVVVDVSQEDPEVQFNWYVDGVEVHNAKTKPREEQFNSTYRVVSVLTVLHQDWLNGKEYKCKVSNKGLPSSIEKTISKAKGQPREPQVYTLPPSQEEMTKNQVSLTCLVKGFYPSDIAVEWESNGQPENNYKTTPPVLDSDGSFFLYSRLTVDKSRWQEGNVFSCSVLHEALHNHYTQKSLSLSLGGGGGSAPTSSSTKKTQLQLEHLLLDLQMILNGINNYKNPKLTAMLTAKFYMPKKATELKHLQCLEEELKPLEEVLNLAQSKNFHLRPRDLISNINVIVLELKGSETTFMCEYADETATIVEFLNRWITFCQSIISTLT

SEQ ID NO: 88 - protein, 18 aa, Artificial Sequence
  Linker1 variant 26
EAAAKAESKYGPPCPPCP

SEQ ID NO: 89 - protein, 605 aa, Artificial Sequence
  GI-101-P26
MDAMLRGLCCVLLLCGAVFVSPSHAVIHVTKEVKEVATLSCGHNVSVEELAQTRIYWQKEKKMVLTMMSGDMNIWPEYKNRTIFDITNNLSIVILALRPSDEGTYECVVLKYEKDAFKREHLAEVTLSVKADFPTPSISDFEIPTSNIRRIICSTSGGFPEPHLSWLENGEELNAINTTVSQDPETELYAVSSKLDFNMTTNHSFMCLIKYGHLRVNQTFNWNTTKQEHFPDNEAAAKAESKYGPPCPPCPAPEAAGGPSVFLFPPKPKDQLMISRTPEVTCVVVDVSQEDPEVQFNWYVDGVEVHNAKTKPREEQFNSTYRVVSVLTVLHQDWLNGKEYKCKVSNKGLPSSIEKTISKAKGQPREPQVYTLPPSQEEMTKNQVSLTCLVKGFYPSDIAVEWESNGQPENNYKTTPPVLDSDGSFFLYSRLTVDKSRWQEGNVFSCSVLHEALHNHYTQKSLSLSLGGGGGSAPTSSSTKKTQLQLEHLLLDLQMILNGINNYKNPKLTAMLTAKFYMPKKATELKHLQCLEEELKPLEEVLNLAQSKNFHLRPRDLISNINVIVLELKGSETTFMCEYADETATIVEFLNRWITFCQSIISTLT

SEQ ID NO: 90 - protein, 23 aa, Artificial Sequence
  Linker1 variant 27
EAAAKEAAAKAESKYGPPCPPCP

SEQ ID NO: 91 - protein, 610 aa, Artificial Sequence
  GI-101-P27
MDAMLRGLCCVLLLCGAVFVSPSHAVIHVTKEVKEVATLSCGHNVSVEELAQTRIYWQKEKKMVLTMMSGDMNIWPEYKNRTIFDITNNLSIVILALRPSDEGTYECVVLKYEKDAFKREHLAEVTLSVKADFPTPSISDFEIPTSNIRRIICSTSGGFPEPHLSWLENGEELNAINTTVSQDPETELYAVSSKLDFNMTTNHSFMCLIKYGHLRVNQTFNWNTTKQEHFPDNEAAAKEAAAKAESKYGPPCPPCPAPEAAGGPSVFLFPPKPKDQLMISRTPEVTCVVVDVSQEDPEVQFNWYVDGVEVHNAKTKPREEQFNSTYRVVSVLTVLHQDWLNGKEYKCKVSNKGLPSSIEKTISKAKGQPREPQVYTLPPSQEEMTKNQVSLTCLVKGFYPSDIAVEWESNGQPENNYKTTPPVLDSDGSFFLYSRLTVDKSRWQEGNVFSCSVLHEALHNHYTQKSLSLSLGGGGGSAPTSSSTKKTQLQLEHLLLDLQMILNGINNYKNPKLTAMLTAKFYMPKKATELKHLQCLEEELKPLEEVLNLAQSKNFHLRPRDLISNINVIVLELKGSETTFMCEYADETATIVEFLNRWITFCQSIISTLT

SEQ ID NO: 92 - protein, 33 aa, Artificial Sequence
  Linker1 variant 28
EAAAKEAAAKEAAAKEAAAKAESKYGPPCPPCP

SEQ ID NO: 93 - protein, 620 aa, Artificial Sequence
  GI-101-P28
MDAMLRGLCCVLLLCGAVFVSPSHAVIHVTKEVKEVATLSCGHNVSVEELAQTRIYWQKEKKMVLTMMSGDMNIWPEYKNRTIFDITNNLSIVILALRPSDEGTYECVVLKYEKDAFKREHLAEVTLSVKADFPTPSISDFEIPTSNIRRIICSTSGGFPEPHLSWLENGEELNAINTTVSQDPETELYAVSSKLDFNMTTNHSFMCLIKYGHLRVNQTFNWNTTKQEHFPDNEAAAKEAAAKEAAAKEAAAKAESKYGPPCPPCPAPEAAGGPSVFLFPPKPKDQLMISRTPEVTCVVVDVSQEDPEVQFNWYVDGVEVHNAKTKPREEQFNSTYRVVSVLTVLHQDWLNGKEYKCKVSNKGLPSSIEKTISKAKGQPREPQVYTLPPSQEEMTKNQVSLTCLVKGFYPSDIAVEWESNGQPENNYKTTPPVLDSDGSFFLYSRLTVDKSRWQEGNVFSCSVLHEALHNHYTQKSLSLSLGGGGGSAPTSSSTKKTQLQLEHLLLDLQMILNGINNYKNPKLTAMLTAKFYMPKKATELKHLQCLEEELKPLEEVLNLAQSKNFHLRPRDLISNINVIVLELKGSETTFMCEYADETATIVEFLNRWITFCQSIISTLT

SEQ ID NO: 94 - protein, 18 aa, Artificial Sequence
  Linker1 variant 29
GGGGSAESKYGPPCPPCP

SEQ ID NO: 95 - protein, 605 aa, Artificial Sequence
  GI-101-P29
MDAMLRGLCCVLLLCGAVFVSPSHAVIHVTKEVKEVATLSCGHNVSVEELAQTRIYWQKEKKMVLTMMSGDMNIWPEYKNRTIFDITNNLSIVILALRPSDEGTYECVVLKYEKDAFKREHLAEVTLSVKADFPTPSISDFEIPTSNIRRIICSTSGGFPEPHLSWLENGEELNAINTTVSQDPETELYAVSSKLDFNMTTNHSFMCLIKYGHLRVNQTFNWNTTKQEHFPDNGGGGSAESKYGPPCPPCPAPEAAGGPSVFLFPPKPKDQLMISRTPEVTCVVVDVSQEDPEVQFNWYVDGVEVHNAKTKPREEQFNSTYRVVSVLTVLHQDWLNGKEYKCKVSNKGLPSSIEKTISKAKGQPREPQVYTLPPSQEEMTKNQVSLTCLVKGFYPSDIAVEWESNGQPENNYKTTPPVLDSDGSFFLYSRLTVDKSRWQEGNVFSCSVLHEALHNHYTQKSLSLSLGGGGGSAPTSSSTKKTQLQLEHLLLDLQMILNGINNYKNPKLTAMLTAKFYMPKKATELKHLQCLEEELKPLEEVLNLAQSKNFHLRPRDLISNINVIVLELKGSETTFMCEYADETATIVEFLNRWITFCQSIISTLT

SEQ ID NO: 96 - protein, 23 aa, Artificial Sequence
  Linker1 variant 30
GGGGSGGGGSAESKYGPPCPPCP

SEQ ID NO: 97 - protein, 610 aa, Artificial Sequence
  GI-101-P30
MDAMLRGLCCVLLLCGAVFVSPSHAVIHVTKEVKEVATLSCGHNVSVEELAQTRIYWQKEKKMVLTMMSGDMNIWPEYKNRTIFDITNNLSIVILALRPSDEGTYECVVLKYEKDAFKREHLAEVTLSVKADFPTPSISDFEIPTSNIRRIICSTSGGFPEPHLSWLENGEELNAINTTVSQDPETELYAVSSKLDFNMTTNHSFMCLIKYGHLRVNQTFNWNTTKQEHFPDNGGGGSGGGGSAESKYGPPCPPCPAPEAAGGPSVFLFPPKPKDQLMISRTPEVTCVVVDVSQEDPEVQFNWYVDGVEVHNAKTKPREEQFNSTYRVVSVLTVLHQDWLNGKEYKCKVSNKGLPSSIEKTISKAKGQPREPQVYTLPPSQEEMTKNQVSLTCLVKGFYPSDIAVEWESNGQPENNYKTTPPVLDSDGSFFLYSRLTVDKSRWQEGNVFSCSVLHEALHNHYTQKSLSLSLGGGGGSAPTSSSTKKTQLQLEHLLLDLQMILNGINNYKNPKLTAMLTAKFYMPKKATELKHLQCLEEELKPLEEVLNLAQSKNFHLRPRDLISNINVIVLELKGSETTFMCEYADETATIVEFLNRWITFCQSIISTLT

SEQ ID NO: 98 - protein, 33 aa, Artificial Sequence
  Linker1 variant 31
GGGGSGGGGSGGGGSGGGGSAESKYGPPCPPCP

SEQ ID NO: 99 - protein, 620 aa, Artificial Sequence
  GI-101-P31
MDAMLRGLCCVLLLCGAVFVSPSHAVIHVTKEVKEVATLSCGHNVSVEELAQTRIYWQKEKKMVLTMMSGDMNIWPEYKNRTIFDITNNLSIVILALRPSDEGTYECVVLKYEKDAFKREHLAEVTLSVKADFPTPSISDFEIPTSNIRRIICSTSGGFPEPHLSWLENGEELNAINTTVSQDPETELYAVSSKLDFNMTTNHSFMCLIKYGHLRVNQTFNWNTTKQEHFPDNGGGGSGGGGSGGGGSGGGGSAESKYGPPCPPCPAPEAAGGPSVFLFPPKPKDQLMISRTPEVTCVVVDVSQEDPEVQFNWYVDGVEVHNAKTKPREEQFNSTYRVVSVLTVLHQDWLNGKEYKCKVSNKGLPSSIEKTISKAKGQPREPQVYTLPPSQEEMTKNQVSLTCLVKGFYPSDIAVEWESNGQPENNYKTTPPVLDSDGSFFLYSRLTVDKSRWQEGNVFSCSVLHEALHNHYTQKSLSLSLGGGGGSAPTSSSTKKTQLQLEHLLLDLQMILNGINNYKNPKLTAMLTAKFYMPKKATELKHLQCLEEELKPLEEVLNLAQSKNFHLRPRDLISNINVIVLELKGSETTFMCEYADETATIVEFLNRWITFCQSIISTLT

SEQ ID NO: 100 - protein, 35 aa, Artificial Sequence
  Linker variant 32
GSGGGGSGGGGSGGGGSAESKYGPPCPPCPGGGGS

SEQ ID NO: 101 - protein, 404 aa, Artificial Sequence
  GI-101-P32
MDAMLRGLCCVLLLCGAVFVSPSHAVIHVTKEVKEVATLSCGHNVSVEELAQTRIYWQKEKKMVLTMMSGDMNIWPEYKNRTIFDITNNLSIVILALRPSDEGTYECVVLKYEKDAFKREHLAEVTLSVKADFPTPSISDFEIPTSNIRRIICSTSGGFPEPHLSWLENGEELNAINTTVSQDPETELYAVSSKLDFNMTTNHSFMCLIKYGHLRVNQTFNWNTTKQEHFPDNGGGGSGGGGSGGGGSGGGGSAESKYGPPCPPCPGGGGSAPTSSSTKKTQLQLEHLLLDLQMILNGINNYKNPKLTAMLTAKFYMPKKATELKHLQCLEEELKPLEEVLNLAQSKNFHLRPRDLISNINVIVLELKGSETTFMCEYADETATIVEFLNRWITFCQSIISTLT

SEQ ID NO: 102 - protein, 70 aa, Artificial Sequence
  Linker variant 33
GSGGGGSGGGGSGGGGSAESKYGPPCPPCPGGGGSGGGGSGGGGSGGGGSGGGGSGGGGSGGGGSGGGGS

SEQ ID NO: 103 - protein, 439 aa, Artificial Sequence
  GI-101-P33
MDAMLRGLCCVLLLCGAVFVSPSHAVIHVTKEVKEVATLSCGHNVSVEELAQTRIYWQKEKKMVLTMMSGDMNIWPEYKNRTIFDITNNLSIVILALRPSDEGTYECVVLKYEKDAFKREHLAEVTLSVKADFPTPSISDFEIPTSNIRRIICSTSGGFPEPHLSWLENGEELNAINTTVSQDPETELYAVSSKLDFNMTTNHSFMCLIKYGHLRVNQTFNWNTTKQEHFPDNGGGGSGGGGSGGGGSGGGGSAESKYGPPCPPCPGGGGSGGGGSGGGGSGGGGSGGGGSGGGGSGGGGSGGGGSAPTSSSTKKTQLQLEHLLLDLQMILNGINNYKNPKLTAMLTAKFYMPKKATELKHLQCLEEELKPLEEVLNLAQSKNFHLRPRDLISNINVIVLELKGSETTFMCEYADETATIVEFLNRWITFCQSIISTLT

SEQ ID NO: 104 - protein, 5 aa, Artificial Sequence
  Linker variant 34
GGGGS

SEQ ID NO: 105 - protein, 371 aa, Artificial Sequence
  GI-101-P34
MDAMLRGLCCVLLLCGAVFVSPSHAVIHVTKEVKEVATLSCGHNVSVEELAQTRIYWQKEKKMVLTMMSGDMNIWPEYKNRTIFDITNNLSIVILALRPSDEGTYECVVLKYEKDAFKREHLAEVTLSVKADFPTPSISDFEIPTSNIRRIICSTSGGFPEPHLSWLENGEELNAINTTVSQDPETELYAVSSKLDFNMTTNHSFMCLIKYGHLRVNQTFNWNTTKQEHFPDNGGGGSAPTSSSTKKTQLQLEHLLLDLQMILNGINNYKNPKLTAMLTAKFYMPKKATELKHLQCLEEELKPLEEVLNLAQSKNFHLRPRDLISNINVIVLELKGSETTFMCEYADETATIVEFLNRWITFCQSIISTLT

SEQ ID NO: 106 - protein, 40 aa, Artificial Sequence
  Linker variant 35
GGGGSGGGGSGGGGSGGGGSGGGGSGGGGSGGGGSGGGGS

SEQ ID NO: 107 - protein, 406 aa, Artificial Sequence
  GI-101-P35
MDAMLRGLCCVLLLCGAVFVSPSHAVIHVTKEVKEVATLSCGHNVSVEELAQTRIYWQKEKKMVLTMMSGDMNIWPEYKNRTIFDITNNLSIVILALRPSDEGTYECVVLKYEKDAFKREHLAEVTLSVKADFPTPSISDFEIPTSNIRRIICSTSGGFPEPHLSWLENGEELNAINTTVSQDPETELYAVSSKLDFNMTTNHSFMCLIKYGHLRVNQTFNWNTTKQEHFPDNGGGGSGGGGSGGGGSGGGGSGGGGSGGGGSGGGGSGGGGSAPTSSSTKKTQLQLEHLLLDLQMILNGINNYKNPKLTAMLTAKFYMPKKATELKHLQCLEEELKPLEEVLNLAQSKNFHLRPRDLISNINVIVLELKGSETTFMCEYADETATIVEFLNRWITFCQSIISTLT

SEQ ID NO: 108 - protein, 233 aa, Artificial Sequence
  CD80 variant 36
MDAMLRGLCCVLLLCGAVFVSPSHAVIHVTKEVKEVATLSCGHNVSVEELAQTRIYWQKEKKMVLTMMSGDMNIWPEYKNRTIFDITNNLSIVILALRPSDEGTYECVVLKYEEDAFKREHLAEVTLSVKADFPTPSISDFEIPTSNIRRIICSASGGFPEPHLSWLENGEELNAINTTVSQDPETELYAVSSKLDFNMTTNHSFMCLIKYGHLRVNQTFNWNTTKQEHFPDN

SEQ ID NO: 109 - protein, 233 aa, Artificial Sequence
  CD80 variant 37
MDAMLRGLCCVLLLCGAVFVSPSHAVIHVTKEVKEVATLSCGHNVSVEELAQTRIYWQKEKKMVLTMMSGDMNIWPEYKNRTIFDITNNLSIVILALRPSDEGTYECVVLKYEEDAFEREHLAEVTLSVKADFPTPSISDFEIPTSNIRRIICSASGGFPEPHLSWLENGEELNAINTTVSQDPETELYAVSSKLDFNMTTNHSFMCLIKYGHLRVNQTFNWNTTKQEHFPDN

SEQ ID NO: 110 - protein, 233 aa, Artificial Sequence
  CD80 variant 38
MDAMLRGLCCVLLLCGAVFVSPSHAVIHVTKEVKEVATLSCGLNVSVEELAQTDILWHKEGKIVLAMRSGDTNIWPEYKNRTIFDITNNLSIVILALRPSDEGTYVCVVRKYENDTPVLEHLAEVTLSVKADFPTPSISDFEIPTSNIRRIICSASGGFPEPHLSWLENGEELSAINTTVSQDPETELYAVSSKLDFNMTTNHSFMCLIKYGHLRVNQTFNWNTTKQEHFPDN

SEQ ID NO: 111 - protein, 233 aa, Artificial Sequence
  CD80 variant 39
MDAMLRGLCCVLLLCGAVFVSPSHAVIHVTKEVKEVGTLSCGHNVSVEELAQTDILWHKEGKIVLAMRSGDTNIWPEYKNRTIFDITNNLSIAILALRPSDEGTYVCVVRKYENDTPVLEHRAEVTLSVKADFPTPSISDFEIPTSNIRRIICSASGGFPEPHLSWLENGEELNAINTTVSQDPETELYAVSSKLDFNMTTNHSFMCHIKYGHLRVNQTFNWNTTKQEHFPDN

SEQ ID NO: 112 - protein, 233 aa, Artificial Sequence
  CD80 variant 40
MDAMLRGLCCVLLLCGAVFVSPSHAVIHVTKEVKEVGTLSCGLNVSAEELAQTRIYWQKEKKMVLTMMSGDMNIWPEYKNRTIFDITNSLSIAILALRPSDEGTYECVVLKYEKDAFKREHLAEVTLSVKADFPTPSISDFEIPTSNIRRIICSASGGFPEPHLSWLENGEELNAINTTVSQDPETELYAVSSKLDFNMTTNHSFMCLIKYGHLRVNQTFNWNTTKQEHFPDN

SEQ ID NO: 113 - protein, 233 aa, Artificial Sequence
  CD80 variant 41
MDAMLRGLCCVLLLCGAVFVSPSHAVIHVTKEVKEVGTLSCGLNVSAEELAQTRIYWQKEKKMVLTMMSGDMNIWPEYKNRTIFDITNSLSIMILALRPSDEGTYECVVLKYEKDAFKREHLAEVTLSVKADFPTPSISDFEIPTSNIRRIICSASGGFPEPHLSWLENGEELNAINTTVSQDPETELYAVSSKLDFNMTTNHSFMCLIKYGHLRVNQTFNWNTTKQEHFPDN

SEQ ID NO: 114 - protein, 130 aa, Artificial Sequence
  CD80 variant 42
MDAMLRGLCCVLLLCGAVFVSPSHAVIHVTKEVKEVATLSCGHNVSVEELAQTRIYWQKEKKMVLTMMSGDMNIWPEYKNRTIFDITNNLSIVILALRPSDEGTYECVVLKYEEDAFKREHLAEVTLSVK

SEQ ID NO: 115 - protein, 133 aa, Artificial Sequence; identical to SEQ ID NO: 23
  hIL2v_3M